European Patent Application EP 4 296 359 A1, published December 27, 2023. Title: Composition for degrading trypsin or TMPRSS2. Applicant: RIKEN Keio University. The sequence listing filed with the application follows.

SEQUENCE LISTING (178 sequences)

SEQ ID NO: 1 - DNA, 3792 bp, Paraprevotella clara
atgaaaaaaaaatcttgtttggtgttcctctttctattgggaatactatggaatgtacaagtccacgctgacggcgtgagccaacctacgttccataccttcaagttcacagaccaagctacactccaaaacatgtccgacaatgggaaatgggctgtagctttcggtacgaacggtaacagtgtggaagattttccgaagctcatagacttggctacggacaaggctaccgaacttttgagcgaaagcggaaccgcattaggcaacggcgcctacgatgtcaataacgagggaactctcgtagtaggacgatatgaaggcaatccggccgtttggaccaaaaccaataacaaatggacagtacttcctgttcctacgggatgggacggtggtttagttaacgccattactcccgacggaaagtgggccataggtagggccaccaaaggtcagtatgacgaaactcccgtactgtgggatatgagtaaaggcggtataatcacagaaacgcctaatatcccggtaaaagacatgaccggactagaccagcaccaaagccgctttgtaggcatttccgctgacggacgttatatcgtaggttgcctgtctttcagctatatccagcctatcgcttgttgttattacgtctatgatcgggataagcaaacatataaattcatcggattcgatgtagatgagaattacaaatggactccgttggctcagaatctggcctttatcgatgatgcacgtatcagcaacaacggaaagtatataacgggtactgcttatatggtaaaagaaggaaatgccgaatacaaaactccttttctttatgacgtcgaagccggttctttctctatttacgaccagaatcaggatcaaggtctcatcggactatgttgtgataacgagggtcatgtgttcggtgcttcaccttcagacagtccggcacgtgaatggagcatacgcgtaggccaatactggtacagcctaacccaaatcctgaaacagcattacaatatagacttcaatacagcttcggggtttgaaaatagcggcactccgattgcccttaatgtagaagggactaaaatcgccgttttcgtctataaaggtgaaagttatatactggagatgcctcaatcgctcgttgaactgaccaatgaaattgatttattggccaactattccgtcagcccggaggaaggttcacaattctctgccctgaaatcactaagcctcacttttgaccgcgacattgaagtgacaggaaagagcagtgccgtaatcttaaaagacgaaaacgggaacaaagtaacaagttcagtaacgttcaaacgtaacgccaataacagcaaaatcgtcgatattagtttccgtggcgcaaacctcgaagacggtaaaaaatatactgtttctgtcccggctggttccatcgttattaatggtgatgccgagaaggcctgcaaggaaattaacattagctacaccggacgggccaataagccagtcgcacctactagcattgcaccggttgacaactcaaccctatcattgttgaacttctctacgaaccctatcatcattaattttgatgcaggaatcgccttgaccgacacggcttacgccgcagtttaccgcaataacgaaacagagccgatgtgcgaactgaaaatggctgtgtcctctctcgacagtaaacaattaggcgtgtacccgtctgccggacaatatttgtataagggtaatgagtattacgtaaaaatcaaggcaggatcagtcacggacgttttaggtagcaatccgaacgaagccatcaacctgcactacacgggtaactatgaacgtgaaatcaactacgacgatgtaacattgttcaaagacgattttaacaacggtttgggccaattcctcttctatgaaggagataaacgcgaaccggtggaaagcatggcccaatggggattcactgcgactacaactccttggagcatcgtatgggatgaggacaacaccagcgatttggcagcagcttcacattccatgtactctccggcaggaaagtctgacgactggatggtaacaacgcaaattttcattccgtctaaccaatgctatttaagatgggagtcacagagttatctcaagagtaaaggagaccgtttgaaaataatggtttgggaatacgaccccgtattgaatgctctgaacgacgatcttatcgctaaattcaagaatgaaggaaaggttatttacgacgaatttgaaaaacctggtgaagacgaaaacaaattagcaggagaatggacttcccacatcgtaaaactggaagagtttaaaggcaaaaacgtatatattgctttcgtgaacgagaacgaagatcaaagtgccatctttatagataatgtggaagtaaccaacgaccagaagtttttggtgggtttgaccaacgaaacctccgtggtaaaccaaaaagaaattaaaatcagtggccgtatcagtatcaatgctttggaagatacttatcagagcgtacacattatcatgaaagacgctaatggtaacgccatagatgaaatcagcgaatctggtctctctttaaagaatggtgacaagtatgactttgctttccaaaaagctctcccgctaagcgtaggcatcgcaaacaagttcacattggatatcactttagatgatgaagaaaaaacaacaggatattctatcaagaatctggctttcgcaccgaccaagcgtttggtgatagaagaatttacaggtacggattgcccgaactgtccgctcggaattctggctttgggcaacatggagaaaatgtttggcgaccaaatcatccccatggctatccacacttacgatggcgacatctactcgaccaaagaacttgaagagtattccgcgttcctgaacttcagtggtgctcccagtggcgtggttaaccgtcagggcggagctacccccgttccttcttatccaatggccagcgttaaaaacacagaaggaaaagtgaattatatattcacaaacggttcggatttatggttagaccaggccgagaaagaattcaaagtggctgcagatgccgaactgaacatcacggcgaagtatcaggacggcaaaatcgtagtgccttgtacctataaatatgcactgaatgcgacagatctaaacgtaagtttgttcatggctattctggaagataacttaacccgttatcaatgtaacaacttgggaggtacttctgacccgaatctcggagaatggggattgggcggccagtacgctgccagtgttgtggcaccttacacgttcaacgatgtagttcgcagcatacccagtgcttactatggtgtaagcggtctgattccttcttccgtaacagccggtgaggagaatacaactagcctggacttaaatatcccggaaaatgtcattgacctcacgaactgtaaagttgtatgtatgatgatcgatgccaacacgggaaacatcatcaatgcagccagagctgacatcaatacagacgattataattccatcgaacaaacaaaagcagacgaaagtatctccgtgaatgctgacaacaacaccatccacattaatgccggcacaacggcacaagttacagtgtacagtgtagacggaagtgttctcgaccaagttgttatcgaaggagaaggcagcctgaagctgcaaggccataagggtatcgtcttggttgaggtaacgaccgagaatactcgtgttgtgaagaaagtattcgtaaaataa

SEQ ID NO: 2 - DNA, 3084 bp, Paraprevotella clara
atgagagagaaactttacacgaaatggaagggaggcctgaataggctttgttttcttcttatgtgtttttgttggactacggttcagtcatgggccgttggtgaagatttacatttaaccattgaaaatggtaagacgtatgaatttgaagctttcaacagttattatcttacttatgtagccacggctaacggacaattatcattgtatcaaaccggtggagacttttgtcgtcagtatacagataacacttttgaaacggaattgccttctacccctcagtatgttaatgagggaaaacttgtagaagtgaaggttgagtcaggtaagacttattatttcttgactcgaggtttaagtaaaggagaactgaccgttactttcggagaaaaagcaactccacttgaattactttcgctctccaaagaagagggaacgacattgaatctttctattgataccctcttaggcttcactttcaatagaatggtaaaagtaggaaattgcacattgtcttccgggtcggtaatcggaaacttgaccgcttcgacgcatgattatggtttcaccgtttccattaaagatgtgttgtataaatggttgaaggagggtaatgtaaaagccggagatgaagtcgttttgactgtaactggattatgtaatgccaatgacgagagcgacaaatacaatggtaatggcgtgctgacggtgaaatatattgcaggagcgttgcctgccgagctggttagcgttgcgaactcacccgaagagatgaatttcctgtcttattacctgcctactgatgaaagggggttggttactttgactttcaaccgttcgatgggcgaagatgctacggcaaaattattctatggcgatatagaaggttcaaatgtctatacggaaagtcttccggtgaaggtgaaagatactcagttgattgtagacctccgtggaaaacgtcgtttgccatctgatatgttaccgaatgccagtgctgatgtgtgggaacagtataaaaccatttccttaaaggttagcaatgtgagggacgcggaaggaaattatgccatgtctacctctcagggtaccacaggttcgtatgcttttaattatacaatagaagctgttgagtttgatatcgctcgtcagtttacaccagatgaaggcacatctttggatgattatccgacaatagaactttggattcgggaagacgattcgtttacttatgagggtgtagatttcacttatagcgtgaatggaaaacctgagacggtatttgtacccatcagccagattacgaaaaaagactctccagacggagatggtgtactattgacgattccggtgccgaataaagcggcggatgagaattcagatgtcgtagtttctttgaataatttgaaagcggccgatggtgcggattattcagaagattttacgataatatataaaacgtcaggaaagagtatggcagggcttgagatagaatctgtgtctcctgctgatggagcagctatcgcggctttagaagctggttcgtttctggaattgtctaccaatatgaatgatcgtgtaggatatgtatggtttagaatagatgaccagaacccgaaggatcctgatcaggcttgtgttaagacgatgacatcgatgaagaaagagacggttgagggaaaagtttctttccggacagaaataattcgtagtgtgactttctttgaagggcatacttataaagttactttcaatgcttatgcttcggagagcgattatcagcacggtgcagatgctcttggtgttatgactgtgacttacactggtacaactccggaatttaagtttagtccggttaagtttgtaggaataacgccggatcctgattatactgtaatttcagacgtaagccagaatgaatttacgttgacttttgacggtcctgtagtattgaatcatgaaaatgcttttgtagtatacggtcagggaatgaattatccatttgaaagtatcgagtcgaatgaagacggtacggaatggacggtaaaggcatccttggaaaaattaatggaaatgggtatgatgcctcgattgtctatgagctttatgccggtggataaagacggaatgttagttgaaggtaatgccggtaaagatgcgacaagttatttgaattttgcctatgattgtacgattggtataccagatttgcaagtgagtccggaaagcggttctaaagtggaaagtttgaaagagatcatagtaggatgtaaagatatcatggacgacaatggtgaggtgatatttcaaggtggtatcagcgaatcttatatggcggccgaaaagatcattttgtataagaacggacgtgagccggttgcaacggtaacgagtatcgaacctattataccggaggaccaagaggataattacttctatgttcctgtggaaatgaaattaacattggatactgaaattacagataacggtaattatcgtttgcacattcctgccaactactttatattgggaacaggtatgtctaatgtaaacagtaaagaaacaagtgtgctgtatactatcgaccagccgattaagataacggttacgccagagaataactctacggtagaaagcctgaaagaaattactatcgaatgtgaatcaggtatagatgtgccgagtatgggtacaattcaattattgaatgctcagaatgaggtggtagcttcggcaacgggtgaggattgcgaattgttgttacccgaaggtgccggtccttgggatccttatactggtgtgacaattaaattggatcaagaggtgacagagaaaggtacatataagttggttattcctgaaggattcttctatttgggtgaaaactatgaaaattcggacgaaatgacgtttacttattcgattaatgccagtggtattcattcgattggtactgagtctaagggagtagtcgtttatactgtagacggtaaatttatcttaaagtcgagcgatgccaaagacgtgaagaatctgaagaaaggtttgtacattgtgaacggtaagaagatgatggtaaaataa

SEQ ID NO: 3 - DNA, 1483 bp, Paraprevotella clara
gatgaacgctagctacaggcttaacacatgcaagtcgaggggcagcatgrrcycagctttgctgggtttgatggcgaccggcgcacgggtgagtaacgcgtatccaacctgccctttactccgggatagtctcctgaaagggagtttaataccggatgtgtttgtctttccgcatgggagcgacaaataaagattgattggtaaaggatggggatgcgtcccattagctrgttggcggggtaacggcccaccaaggcracgatgggtaggggttctgagaggaaggtcccccacattggaactgagacacggtccaaactcctacgggaggcagcagtgaggaatattggtcaatgggcgagagcctgaaccagccaagtagcgtgaaggacgacggccctacgggttgtaaacttcttttataagggaataaagttcgccacgcgtggtgttttgtatgtaccttatgaataagcatcggctaattccgtgccagcagccgcggtaatacggaagatgcgagcgttatccggatttattgggtttaaagggagcgtaggcgggcttttaagtcagcggtcaaatgtcacggctcaaccgtggccagccgttgaaactgtaagccttgagtctgcacagggcacatggaattcgtggtgtagcggtgaaatgcttagatatcacgaagaactccgatcgcgaaggcattgtgccggggcagcactgacgctgaggctcgaaagtgcgggtatcaaacaggattagataccctggtagtccgcacggtaaacgatgaatgctcgctatgggcgatayawtgtccgtggccaagcgaaagcgttaagcattccacctggggagtacgccggcaacggtgaaactcaaaggaattgacgggggcccgcacaagcggaggaacatgtggtttaattcgatgatacgcgaggaaccttacccgggcttgaattgcaggtgcatgagtcagagatgattctttccttcgggactcctgtgaaggtgctgcatggttgtcgtcagctcgtgccgtgaggtgtcggcttaagtgccataacgagcgcaacccttctccccagttgccatcgggtaatgccgggccctctggggacactgccatcgtaagatgcgaggaaggtggggatgacgtcaaatcagcacggcccttacgtccggggctacacacgtgttacaatggggggtacagagggccgctgtccggtgacggttggccaatccctaaaacccctctcagttcggactggagtctgcaacccgactccacgaagctggattcgctagtaatcgcgcatcagccatggcgcggtgaatacgttcccgggccttgtacacaccgcccgtcaagccatgaaagccgggggtgcctgaagtccgtgaccgcgagggtcggcctagggtaaaactggtgattggggctaagtcgtaacaaggtagccgtaccggaagg

SEQ ID NO: 4 - DNA, 1482 bp, Paraprevotella xylaniphila
gatgaacgctagctacaggcttaacacatgcaagtcgaggggcagcatgagctcagttattctgggtttgatggcgaccggcgcacgggtgagtaacgcgtatccaacctgccctttacccggggatagccttctgaaaggaagtttaatacccgatgatttcgtttagtcgcatgacttgatgaataaagattaattggtaaaggatggggatgcgtcccattagcttgttggcggggtaacggcccaccaaggcgacgatgggtaggggttctgagaggaaggtcccccacattggaactgagacacggtccaaactcctacgggaggcagcagtgaggaatattggtcaatgggcgcgagcctgaaccagccaagtagcgtggaggacgacggccctacgggttgtaaactccttttataaggggataaagttggccatgtatggccatttgcaggtaccttatgaataagcatcggctaattccgtgccagcagccgcggtaatacggaagatgcgagcgttatccggatttattgggtttaaagggagcgtaggcgggcagtcaagtcagcggtcaaatggcgcggctcaaccgcgttccgccgttgaaactggcagccttgagtatgcacagggtacatggaattcgtggtgtagcggtgaaatgcttagatatcacgaggaactccgatcgcgcaggcattgtaccggggcattactgacgctgaggctcgaaggtgcgggtatcaaacaggattagataccctggtagtccgcacagtaaacgatgaatgcccgctgtcggcgacatagtgtcggcggccaagcgaaagcgttaagcattccacctggggagtacgccggcaacggtgaaactcaaaggaattgacgggggcccgcacaagcggaggaacatgtggtttaattcgatgatacgcgaggaaccttacccgggcttgaatcgcaggtgcatgggccggagacggccctttccttcgggactcctgcgaaggtgctgcatggttgtcgtcagctcgtgccgtgaggtgtcggcttaagtgccataacgagcgcaacccccctccccagttgccaccgggtaatgccgggcactttggggacactgccaccgcaaggtgcgaggaaggtggggatgacgtcaaatcagcacggcccttacgtccggggcgacacacgtgttacaatggggggtacagagggccgctgcccggtgacggttggccaatccctaaaacccctctcagttcggactggagtctgcaacccgactccacgaagctggattcgctagtaatcgcgcatcagccatggcgcggtgaatacgttcccgggccttgtacacaccgcccgtcaagccatgaaagccgggggtgcctgaagtccgtgaccgcgagggtcggcctagggtaaaaccggtgattggggctaagtcgtaacaaggtagccgtaccggaagg

SEQ ID NO: 5 - protein, 1263 aa, Paraprevotella clara
MKKKSCLVFLFLLGILWNVQVHADGVSQPTFHTFKFTDQATLQNMSDNGKWAVAFGTNGNSVEDFPKLIDLATDKATELLSESGTALGNGAYDVNNEGTLVVGRYEGNPAVWTKTNNKWTVLPVPTGWDGGLVNAITPDGKWAIGRATKGQYDETPVLWDMSKGGIITETPNIPVKDMTGLDQHQSRFVGISADGRYIVGCLSFSYIQPIACCYYVYDRDKQTYKFIGFDVDENYKWTPLAQNLAFIDDARISNNGKYITGTAYMVKEGNAEYKTPFLYDVEAGSFSIYDQNQDQGLIGLCCDNEGHVFGASPSDSPAREWSIRVGQYWYSLTQILKQHYNIDFNTASGFENSGTPIALNVEGTKIAVFVYKGESYILEMPQSLVELTNEIDLLANYSVSPEEGSQFSALKSLSLTFDRDIEVTGKSSAVILKDENGNKVTSSVTFKRNANNSKIVDISFRGANLEDGKKYTVSVPAGSIVINGDAEKACKEINISYTGRANKPVAPTSIAPVDNSTLSLLNFSTNPIIINFDAGIALTDTAYAAVYRNNETEPMCELKMAVSSLDSKQLGVYPSAGQYLYKGNEYYVKIKAGSVTDVLGSNPNEAINLHYTGNYEREINYDDVTLFKDDFNNGLGQFLFYEGDKREPVESMAQWGFTATTTPWSIVWDEDNTSDLAAASHSMYSPAGKSDDWMVTTQIFIPSNQCYLRWESQSYLKSKGDRLKIMVWEYDPVLNALNDDLIAKFKNEGKVIYDEFEKPGEDENKLAGEWTSHIVKLEEFKGKNVYIAFVNENEDQSAIFIDNVEVTNDQKFLVGLTNETSVVNQKEIKISGRISINALEDTYQSVHIIMKDANGNAIDEISESGLSLKNGDKYDFAFQKALPLSVGIANKFTLDITLDDEEKTTGYSIKNLAFAPTKRLVIEEFTGTDCPNCPLGILALGNMEKMFGDQIIPMAIHTYDGDIYSTKELEEYSAFLNFSGAPSGVVNRQGGATPVPSYPMASVKNTEGKVNYIFTNGSDLWLDQAEKEFKVAADAELNITAKYQDGKIVVPCTYKYALNATDLNVSLFMAILEDNLTRYQCNNLGGTSDPNLGEWGLGGQYAASVVAPYTFNDVVRSIPSAYYGVSGLIPSSVTAGEENTTSLDLNIPENVIDLTNCKVVCMMIDANTGNIINAARADINTDDYNSIEQTKADESISVNADNNTIHINAGTTAQVTVYSVDGSVLDQVVIEGEGSLKLQGHKGIVLVEVTTENTRVVKKVFVK

SEQ ID NO: 6 - protein, 1263 aa, Paraprevotella clara
MKKKSCLVFLFLLGILWNVQVHADGVSQPTFHTFKFTDQATLQNMSDNGKWAVAFGTNGNSVEDFPKLIDLATDKATELLSESGTALGNGAYDVNNEGTLVVGRYEGNPAVWTKTNNKWTVLPVPTGWDGGLVNAITPDGKWAIGRATKGQYDETPVLWDMSKGGIITETPNIPVKDMTGLDQHQSRFVGISADGRYIVGCLSFSYIQPIACCYYVYDRDKQTYKFIGFDVDENYKWTPLAQNLAFIDDARISNNGKYITGTAYMVKEGNAEYKTPFLYDVEAGSFSIYDQNQDQGLIGLCCDNEGHVFGASPSDSPAREWSIRVGQYWYSLTQILKQHYNIDFNTVSGFENSGTPIALNVEGTKIAVFVYKGESYILEMPQSLVELTNEIDLLANYSVSPEEGSQFSALKSLSLTFDRDIEVTGKSSAVILKDENGNKVTSSVTFKRNANNSKIVDISFRGANLEDGKKYTVSVPAGSIVINGDAEKACKEINISYTGRANKPVAPTSIAPVDNSTLSLLNFSTNPIIINFDAGIALTDTAYAAVYRNNETEPMCELKMAVSSLDSKQLGVYPSAGQYLYKGNEYYVKIKAGSVTDVLGSNPNEAINLHYTGNYEREINYDDVTLFKDDFNNGLGQFLFYEGDKREPVESMVQWGFTATTTPWSIVWDEDNTSDLAAASHSMYSPAGKSDDWMVTTQIFIPSNQCYLRWESQSYLKSKGDRLKIMVWEYDPVLNALNDDLIAKFKNEGKVIYDEFEKPGEDENKLAGEWTSHIVKLEEFKGKNVYIAFVNENEDQSAIFIDNVEVTNDQKFLVGLTNETSVVNQKEIKISGRISINALEDTYQSVHIIMKDANGNAIDEISESGLSLKNGDKYDFAFQKALPLSVGIANKFTLDITLDDEEKTTGYSIKNLAFAPTKRLVIEEFTGTDCPNCPLGILALGNMEKMFGDQIIPMAIHTYDGDIYSTKELEEYSAFLNFSGAPSGVVNRQGGATPVPSYPMASVKNTEGKVNYIFTNGSDLWLDQAEKEFKVAADAELNITAKYQDGKIVVPCTYKYALNATDLNVSLFMAILEDNLTRYQCNNLGGTSDPNLGEWGLGGQYAASVVAPYTFNDVVRSIPSAYYGVSGLIPSSVTAGEENTTSLDLNIPENIIDLTNCKVVCMMIDANTGNIINAARADINTDDYNSIEQTKADESISVNADNNTIHINAGTTAQVTVYSVDGSVLDQVVIEGEGSLKLQGHKGIVLVEVTTENTRVVKKVFVK

SEQ ID NO: 7 - DNA, 3792 bp, Paraprevotella clara
atgaaaaaaaaatcttgtttggtgttcctctttctattgggaatactatggaatgtacaagtccacgctgacggtgtgagccaacctacgttccataccttcaagttcacagaccaagctacactccagaacatgtccgacaatgggaaatgggctgtagctttcggtacgaacggtaacagtgtggaagattttccgaagctcatagacttggctacggacaaggctaccgaacttttgagcgaaagcggaaccgcattaggcaacggcgcctacgatgtcaataacgagggaactctcgtagtaggacgatatgaaggaaatccggccgtttggaccaaaaccaataacaaatggacagtacttcctgttcctacgggatgggacggtggtttagttaacgccattactcccgacggaaagtgggccataggtagggccaccaaaggtcagtatgacgaaactcccgtactgtgggatatgagtaaaggcggtataatcacagaaacgcctaatatcccggtaaaagacatgaccggactagaccagcaccaaagccgctttgtaggcatttccgctgacggacgttatatcgtaggttgcctgtctttcagctatatccagcctatcgcttgttgttattacgtctatgatcgggataagcaaacatataaattcatcggattcgatgtagatgagaattacaaatggactccgttggctcagaatctggcctttatcgatgatgcacgtatcagcaacaacggaaagtatataacgggtactgcttatatggtaaaagaaggaaatgccgaatacaaaactccttttctttatgacgttgaagccggttccttctctatttacgaccagaaccaggaccaaggtctcatcggactatgttgtgataacgagggtcatgtgttcggtgcttcaccttcagacagtccggcacgtgaatggagcatacgcgtaggccaatactggtacagccttacccaaatcctgaaacagcattacaatatagactttaatacagtttcggggtttgaaaatagcggaactccgattgcccttaatgtagaaggtactaaaatcgccgtcttcgtctataaaggtgaaagttatatactggagatgcctcagtcgctcgttgaactgaccaatgaaattgatttattggccaactattccgtcagcccggaggaaggttcacaattctctgccctgaaatcactaagcctcacttttgaccgcgacattgaagtgacaggaaagagcagtgccgtaatcttaaaagacgaaaacgggaacaaagtaacaagttcagtaacgttcaaacgtaacgccaataacagcaaaatcgtcgatattagtttccgtggcgcaaacctcgaagacggtaaaaaatatactgtttctgtcccggctggttccatcgttattaatggtgatgccgagaaggcctgcaaggaaattaacattagctacaccggacgggccaataagccagtcgcacctactagcattgcaccggttgacaactcaaccctatcattgttgaacttctctacgaaccctatcatcattaattttgatgcaggaatcgccttgaccgacacggcttacgccgcagtttaccgcaataacgaaacagagccgatgtgcgaactgaaaatggctgtgtcctctctcgacagtaaacaattaggcgtgtacccgtctgccggacaatatttgtataagggtaatgagtattacgtaaaaatcaaggcaggatcagtcacggacgttttaggtagcaatccgaacgaagccatcaacctgcactacacgggtaactatgaacgtgaaatcaactacgacgatgtaacattgttcaaagacgattttaacaacggtttgggccaattcctcttctatgaaggagataaacgcgaaccggtggaaagcatggtccaatggggattcactgcgactacaactccttggagcatcgtatgggatgaggacaacaccagcgatttggcagcagcttcacattccatgtactctccggcaggaaagtctgacgactggatggtaacaacgcaaattttcattccgtctaaccaatgctatttaagatgggagtcacagagttatcttaagagtaaaggagaccgtttgaaaataatggtttgggaatacgaccccgtattgaatgctctgaacgacgatcttatcgctaaattcaagaatgaaggaaaggttatttacgacgaatttgaaaaacctggtgaagacgaaaacaaattagcaggagaatggacttcccacatcgtaaaactggaagagtttaaaggcaaaaacgtatatattgctttcgtgaacgagaacgaagatcaaagtgccatctttatagataatgtggaagtaaccaacgaccagaagtttttggtgggtttgaccaacgaaacctccgtggtaaaccaaaaagaaattaaaatcagtggccgtatcagtatcaatgctttggaagatacttatcagagcgtacacattatcatgaaagacgctaatggtaacgccatagatgaaatcagcgaatctggtctctctttaaagaatggtgacaagtatgactttgctttccaaaaagctctcccgctaagcgtaggcatcgcaaacaagttcacattggatatcactttagatgatgaagaaaaaacaacaggatattctatcaagaatctggctttcgcaccgaccaagcgtttggtgatagaagaatttacaggtacggattgcccgaactgtccgctcggaattctggctttgggcaacatggagaaaatgtttggcgaccaaatcatccccatggctatccacacttacgatggcgacatctactcgaccaaagaacttgaagagtattccgcgttcctgaacttcagtggtgctcccagcggagtagtcaatcgtcagggcggagctacccccgttccttcttatccaatggccagcgttaaaaacacagaaggaaaagtgaattatatattcacaaacggttcggatttatggttagaccaggccgagaaagaattcaaagtggctgcagatgccgaactgaacatcacggcgaagtatcaggacggcaaaatcgtagtgccttgtacctataaatatgcactgaatgccacggatctaaatgtaagtttgttcatggcaattctggaagataacttaacccgttatcaatgtaacaacttgggaggtacttctgacccgaatctcggagaatggggattgggcggccagtacgctgccagtgtagtggcaccttacacgttcaacgatgtagttcgcagcatacccagtgcttactatggtgtaagcggtctgattccttcttccgtaacagccggtgaggagaatacgactagtctggacttaaatatcccggaaaatatcattgatctcacaaactgtaaagtagtatgtatgatgatcgatgccaacacgggaaacatcatcaatgcagccagagctgatatcaatacagacgattataattccatcgaacaaacaaaagcagacgaaagtatctccgtgaatgctgacaacaacaccatccacattaatgccggcacaacggcacaagttacggtgtacagtgtagacggaagtgttctcgaccaagttgttatcgaaggagaaggtagcctgaagctgcaaggccataagggtatcgtcttggttgaggtaacgaccgagaatactcgtgttgtgaagaaagtattcgtaaaataa

SEQ ID NO: 8 - protein, 1198 aa, Paraprevotella xylaniphila
MFPKLIDLSSNQVTELLTGEDYSNLTSAAYDVTDDGSMVAGSYDGQPAIYITAQKRWSMLAVPDSCVGGEVTAITPDGHYAVGRGLYANTYMEAVVMWDLQQDGLLLDLSGIPFEDMVGENNNQRRLIGVTPDGNKVLGCISYSYVSPAGIFFFVYDRQTKKCQPIGFDTTTETTEEGPQTVWTPRAEGLYFINSADLSANGRYITGEAYMENDAAKGYVYDIETDKFTLYSDAQDDMPGFTACSNGIVLGATPPTNPYRDWSVRVGEYWYPISLILSQRYGINFSTETNFSNTGTPIATSLDGKKIVVFVAPQKENYILELPETLDAATTDIDLLGNYIVNPKAGSEFSSLKTVTFTFPYEIELLGDKSNVTFTDENGKKTGTILSLKTDDKDLNISFRSTNLQAGVKYTLTLSAGTIAIKGDTERKNKELSVTYTGRDNVPVKMVSATPYENTEVKQLNYTNNPITITFDTQLSLNEDAIGYLYKDDETTPDGTLRLGVTDNKLYVFPVTARNLFKGHNYKVTVPRNAVYDIMGNNGNDSITLHYIGGFEREVSYDNDTLFVEDFNNGFTKTMLYEGDHNKPTEEMQKMDFNDSDNYPWTMVRDEDDPNNYAAASTSLYDPVGRSDDWMVTAHIYIPDDRCYLQFDAQSFRENKKDSLYVLVWVTEDEFSSMNSERIAKFKAECDTIYAGIETPGDYEDFLAGDWTEHTASLQPYAGKNIYIAFVNSNENQSCVFVDNLLVRQDQQFQISVTTDQTVVKAKEIKISGQIRITTPDHTYSTLELTLKDSQGNMVDQISESNLELKENDKYDFSFDKPLPLVIGQENEYTILVQLDEEQSEPHYSVKNLSFQTVKRVVLEEGTGQDCPNCPQGILAIENLEDVYGDLFIPVSLHTYSGDPYGTGFESYAAFLNITGYPSGTVNRTNQVPVGAMTSDENGNATFTSTAHPCWLDYVAAEMEISADANFDIAKAKVEADSTINMTYKYQYALNVKGQNVNLFTVILEDSLIGKQRNSYGSNSDPLLGEWGQGGKYSAATVRNYPFVDVVRGVVGDTFYGTAGYIQPNVEAGKEYTAEATFKLPAKVLKAKNCKIVTMMIDANSGKVINSARAKLDVSDFANAIADIQAEKPNVEIAVVNGGVEITTDAPAQINLYSLNGTLIGTAKSQGFVSLSTNGYRGLTLVKVTTGHQTLVKKVIVK

SEQ ID NO: 9 - DNA, 3597 bp, Paraprevotella xylaniphila
atgtttcccaaacttatcgacttaagctctaaccaagtcacggaactgcttaccggcgaagactactccaacttgacaagcgcggcctatgacgtgacagacgacggtagcatggtggcaggaagctatgacggccaaccggctatctatatcacagcccaaaaacgttggagcatgttggccgtacccgacagctgtgtaggtggagaagtcacagccatcacccccgatggccattacgccgtgggaaggggcctatacgcaaatacttacatggaagctgtcgtcatgtgggatttacaacaggacggcctgcttctcgatttatccggcattccatttgaagacatggtaggcgaaaataacaaccaacgccgtctgataggtgtaacccctgatggaaataaagtattaggctgcatatcatacagctacgtaagccctgccggcatcttcttttttgtatatgaccgccaaaccaagaagtgccagcctatcggtttcgataccacaacagaaacaacagaagaaggccctcaaacggtttggacaccgcgtgccgaaggactttattttatcaactcagccgatctcagtgccaacggacgatatatcacaggcgaagcgtacatggaaaatgatgcagccaaaggttacgtttacgacatagaaacggataaattcaccctatacagcgatgcacaagatgacatgcccggttttacagcatgcagtaatggaatcgtgttgggtgcaacccctccgaccaatccttatcgtgactggagcgtgcgcgtgggagaatattggtatcccatttctttgattctctctcaacgttatggcatcaacttctctacggagactaatttctccaatacaggaacaccgatagccactagcctggatggcaaaaaaatcgttgtattcgtagctccacaaaaagaaaattatattttggaattaccggagaccttggatgcagcaaccacagatattgacttattaggtaactacatcgtcaatccgaaggccggaagtgaattctcgtctcttaaaaccgtcacgtttacattcccctatgaaatagaactattaggagacaaaagcaatgtgacctttacggacgaaaacgggaaaaaaacgggtacgatcttaagtcttaaaacggatgacaaggatttgaatatcagcttccgcagcacaaacctgcaagcaggagtgaaatataccctgaccctttctgccggtactatcgccatcaaaggcgacacggaacgtaaaaacaaagagctctccgtcacttatacaggacgtgataatgttccggtaaaaatggtatctgccactccgtatgaaaacacggaagtaaaacagctgaattacaccaacaatcctataaccataacgttcgacacccaattatccctcaatgaggacgctatcggttacctttacaaagacgacgaaacgaccccggacggcaccttacgtttaggagtcacagacaataaattatatgtgttccctgtcacagcccgcaatttgtttaagggacacaactacaaagtgacggttcctcgcaacgcggtatatgacatcatgggcaataatggtaatgactccatcaccttgcactacatcggcggattcgaacgcgaagtaagttatgacaacgatacactcttcgtagaggatttcaacaacgggttcactaagaccatgttgtatgaaggagaccataataaacccacggaggaaatgcaaaaaatggatttcaacgatagcgataactatccttggaccatggtacgcgatgaagatgatcccaataactatgccgctgcttccacttcgttgtatgaccccgtcgggaggtctgacgactggatggtcacagcgcatatctatatcccggacgacagatgttatttgcaatttgatgcccaaagtttccgggagaataaaaaagatagcctttatgtattggtttgggtaactgaagatgagttttcttcaatgaacagcgaacgtatcgccaagttcaaagccgaatgcgacaccatatatgccggcatcgaaactccgggagactatgaagacttccttgccggagactggacggaacacacggcaagcctacaaccttatgccggcaaaaacatctacatcgcttttgtcaacagcaatgaaaaccaaagttgtgtattcgtagacaaccttttggtgagacaagaccaacagttccaaatcagcgtgaccacagaccaaacggtggtaaaagccaaagagataaaaatcagtggacaaatcagaatcacgacaccagaccacacttactcgaccttggaactgaccttgaaagattctcagggaaacatggtagaccaaattagcgaaagcaacctggaactgaaagaaaatgataagtatgacttctccttcgacaagccattacccttggttatcggccaagaaaacgaatatactatccttgtccaattggatgaagaacaaagtgaacctcactattcagtaaagaacctgtctttccagaccgttaaacgggttgtattggaagaaggtaccggacaggattgtccgaactgtccgcaaggcattctggccattgaaaatctggaagatgtttacggcgacttgttcatccctgtaagccttcatacttattccggtgacccttatggaactggctttgaaagctatgccgcattcctgaacatcacaggatacccttcgggcaccgtcaatcgtaccaatcaagtccctgtgggagccatgacttcggatgagaatggaaatgccaccttcacctctacggcacatccttgttggttagactatgtagctgcagaaatggaaataagcgccgatgcaaacttcgacatcgcaaaggctaaggtagaggcagacagtacaattaacatgacttataaataccaatatgccctaaacgtgaaaggacaaaacgtaaacctctttactgtaatattagaagatagcctgattggcaagcaaagaaactcttatggttccaacagcgacccgcttttaggcgaatggggccagggaggtaaatactctgccgccaccgtacgtaattatcctttcgtagatgtagtgagaggcgtagtcggtgatacattctacggcactgccggttatatccaaccgaatgtcgaggccggtaaggaatatacggccgaagccactttcaagcttcctgcaaaagtcctgaaagctaaaaactgtaagatcgtaaccatgatgatagacgccaacagcggcaaagtcatcaattcggcgcgcgccaaattggatgtatcggattttgctaatgccatagctgacatacaagcagaaaaaccgaatgtcgaaattgcagttgtaaacggtggcgtagagattaccacagatgccccggcacaaattaatttgtatagcctgaacggcactttaatcggaacagccaaaagccaaggctttgtctcattaagcacaaacggataccgtggccttactttggtgaaagtgactaccggacatcaaactttagtgaaaaaagtcatcgtgaagtaa

SEQ ID NO: 10 - protein, 1260 aa, Paraprevotella xylaniphila
MKKGLLKIALSVLGAAFFLCAKAQGVPGASIHPFVFEDVSILTNISNNGKWATAHGTEESKTMFPKLIDLSSNQVTELLTGEDYSNLTSAAYDVTDDGSMVAGSYDGQPAIYITAQKRWSMLAVPDSCVGGEVTAITPDGHYAVGRGLYADTYMEAVVMWDLQQDGLLLDLSGIPFEDMVGENNNQRRLIGVTPDGNKVLGCISYSYVSPAGIFFFVYDRQTKKCQPIGFDTTTETTEEGPQTVWTPRAEGLYFINSANLSANGRYITGEAYMENDAAKGYVYDIETDKFTLYSDAQDDMPGFTACSNGIVLGATPPTNPYRDWSVRVGEYWYPISLILSQRYGINFSTETNFSNTGTPIATSLDGKKIVVFVAPQKENYILELPETLDAATTDIDLLGNYIVNPKAGSEFSSLKTVTFTFPYEIELLGDKSNVTFTDENGKKTGTILSLKTDDKDLNISFRSTNLQAGVKYTLTLSAGTIAIKGDTERKNKELSVTYTGRDNVPVKMVSATPYENTEVKQLNYTNNPITITFDTQLSLNEDAIGYLYKDDETTPDGTLRLGVTDNKLYVFPVTARNLFKGHNYKVTVPRNAVYDIMGNNGNDSITLHYIGGFEREVSYDNDTLFVEDFNNGFTKTMLYEGDHNKPTEEMQKMDFNDSDNYPWTMVRDEDDPNNYAAASTSLYDPVGRSDDWMVTAHIYIPDDRCYLQFDAQSFRENKKDSLYVLVWVTEDEFSSMNSERIAKFKAECDTIYAGIETPGDYEDFLAGDWTEHTASLQPYAGKNIYIAFVNSNENQSCVFVDNLLVRQDQQFQISVTTDQTVVKAKEIKISGQIRITTPDHTYSTLELTLKDSQGNMVDQISESNLELKENDKYDFSFDKPLPLVIGQENEYTILVQLDEEQSEPHYSVKNLSFQTVKRVVLEEGTGQDCPNCPQGILAIENLEDVYGDLFIPVSLHTYSGDPYGTGFESYAAFLNITGYPSGTVNRTNQVPVGAMTSDENGNATFTSTAHPCWLDYVAAEMEISADANFDIAKAKVEADSTINMTYKYQYALNVKGQNVNLFTVILEDSLIGKQRNSYGSNSDPLLGEWGQGGKYSAATVRNYPFVDVVRGVVGDTFYGTAGYIQPNVEAGKEYTAEATFKLPAKVLKAKNCKIVTMMIDANSGKVINSARAKLDVSDFANAIADIQAEKPNVEIAVVNGGVEITTDAPAQINLYSLNGTLIGTAKSQGFVSLSTNGYRGLTLVKVTTGHQTLVKKVIVK

SEQ ID NO: 11 - DNA, 3783 bp, Paraprevotella xylaniphila
atgaagaaaggtctattaaaaattgccctctcagtattaggagcggcgttttttctttgcgcgaaagcgcaaggggttccaggagcctccattcatccgtttgtatttgaagatgtatccatccttactaacatttcaaacaacgggaaatgggctaccgctcatggtacagaggaaagcaaaacgatgtttcccaaacttatcgacttaagctctaaccaagtcacggaactgcttaccggcgaagactactccaacttgacaagcgcggcctatgacgtgacagacgacggtagcatggtggcaggaagctatgacggccaaccggctatctatatcacagcccaaaaacgttggagcatgttggccgtacccgacagctgtgtaggtggagaagtcacagccatcacccccgatggccattacgccgtgggaaggggcctatacgcagatacttacatggaagctgtcgtcatgtgggatttacaacaggacggcctgcttctcgatttatccggcattccatttgaagacatggtaggcgaaaataacaaccaacgccgtctgataggtgtaacccctgatggaaataaagtattaggctgcatatcatacagctacgtaagccctgccggcatcttcttttttgtatatgaccgccaaaccaagaagtgccagcctatcggtttcgataccacaacagaaacaacagaagaaggccctcaaacggtttggacaccgcgtgccgaaggactttattttatcaactcagccaatctcagtgctaacggacgatatatcacaggcgaagcgtacatggaaaatgatgcagccaaaggttacgtttacgacatagaaacggataaattcaccctatacagcgatgcacaagatgacatgcccggttttacagcatgcagtaatggaatcgtgttgggtgcaacccctccgaccaatccttatcgtgactggagcgtgcgcgtgggagaatattggtatcccatttctttgattctctctcaacgttatggcatcaacttctctacggagactaatttttctaatacaggaacaccgatagccactagcctggatggcaaaaaaatcgttgtattcgtagctccacaaaaagaaaattatattttggaattaccggagaccttggatgcagcaaccacagatattgacttattaggtaactacatcgtcaatccgaaggccggaagtgaattctcgtctcttaaaaccgtcacgtttacattcccctatgaaatagaactattaggagacaaaagcaatgtgacctttacggacgaaaacgggaaaaaaacgggtacgatcttaagtcttaaaacggatgacaaggatttgaatatcagcttccgcagcacaaacctgcaagcaggagtgaaatataccctgaccctttctgccggtactatcgccatcaaaggcgacacggaacgtaaaaacaaagagctctccgtcacttatacaggacgtgataatgttccggtaaaaatggtatctgccactccgtatgaaaacacggaagtaaaacagctgaattacaccaacaatcctataaccataacgttcgacacccaattatccctcaatgaggacgctatcggttacctttacaaagacgacgaaacgaccccggacggcaccttacgtttaggagtcacagacaataaattatatgtgttccctgtcacagcccgcaatttgtttaagggacacaactacaaagtgacggttcctcgcaacgcggtatatgacatcatgggcaataatggtaatgactccatcaccttgcactacatcggcggattcgaacgcgaagtaagttatgacaacgatacactcttcgtagaggatttcaacaacgggttcactaagaccatgttgtatgaaggagaccataataaacccacggaggaaatgcaaaaaatggatttcaacgatagcgataactatccttggaccatggtacgcgatgaagatgatcccaataactatgccgctgcttccacttcgttgtatgaccccgtcgggaggtctgacgactggatggtcacagcgcatatctatatcccggacgacagatgttatttgcaatttgatgcccaaagtttccgggagaataaaaaagatagcctttatgtattggtttgggtaactgaagatgagttttcttcaatgaacagcgaacgtatcgccaagttcaaagccgaatgcgacaccatatatgccggcatcgaaactccgggagactatgaagacttccttgccggagactggacggaacacacggcaagcctacaaccttatgccggcaaaaacatctacatcgcttttgtcaacagcaatgaaaaccaaagttgtgtattcgtagacaaccttttggtgagacaagaccaacagttccaaatcagcgtgaccacagaccaaacggtggtaaaagccaaagagataaaaatcagtggacaaatcagaatcacgacaccagaccacacttactcgaccttggaactaaccttgaaagattctcagggaaacatggtagaccaaattagcgaaagcaacctggaactgaaagaaaatgataagtatgacttctccttcgacaagccattacccttggttatcggccaagaaaacgaatatactatccttgtccaattggatgaagaacaaagtgaacctcactattcagtaaagaacctgtctttccagaccgttaaacgggttgtattggaagaaggtaccggacaggattgtccgaactgtccgcaaggcattctggccattgaaaatctggaagatgtttacggcgacttgttcatccctgtaagccttcatacttattccggtgacccttatggaactggctttgaaagctatgccgcattcctgaacatcacaggatacccttcgggcaccgtcaatcgtaccaatcaagtccctgtgggagccatgacttcggatgagaatggaaatgccaccttcacctctacggcacatccttgttggttagactatgtagctgcagaaatggaaataagcgccgatgcaaacttcgacatcgcaaaggctaaggtagaggcagacagtacgattaacatgacttataaataccaatatgccctaaacgtgaaaggacaaaacgtaaacctctttactgtaatattagaagatagcctgattggcaagcaaagaaactcttatggttccaacagcgacccacttttaggcgaatggggccagggaggtaaatactctgccgccaccgtacgtaattatcctttcgtagatgtagtgagaggcgtagtcggtgatacattctacggcactgccggttatatccaaccgaatgtcgaggccggtaaggaatatacggccgaagccactttcaagcttcctgcaaaagtcctgaaagctaaaaactgtaagatcgtaaccatgatgatagacgccaacagcggcaaagtcatcaattcggcgcgcgccaaattggatgtatcggattttgctaatgccatagctgacatacaagcagaaaaaccgaatgtcgaaattgcagttgtaaacggtggcgtagagattaccacagatgccccggcacaaattaatttgtatagcctgaacggcactttaatcggaacagccaaaagccaaggctttgtctcattaagcacaaacggataccgtggccttactttggtgaaagtgactaccggacatcaaactttagtgaaaaaagtcatcgtgaagtaa

SEQ ID NO: 12 - protein, 1242 aa, Prevotella rara
MGLLWAIPSSAQEAQLTTVSFPKAAAFTSLSDNGLWATAAGVNDDDQSKYAYPYLINVETGALTELWVEADLIKSLEATDVTNDGKIIVGTYDSKPAYYDMNQGKWITLQSENPGKATSVTPDGKYISGWSNSGSFSGDAYVETPLLWEKQSDGTYRAIDVYAELPNFPKKTKLGTNTQQVRIDNVSPDGNILSGIINFVTPATVCYYVYNKTTQECKYVDNALGEVPDETFVDESTMSNNGKYLTGIVQVAGGSYISSYLYNTSDNSCILYNTESEEQDRAGSAVSNTGVVFACSPAVNPVRSAYVRVGSLWYGIDEILSGRYDMNFYERTGYDFTGTIQGVSDDEKTIIGMSETKTKGYIIRLPETISEAASSVNPLGTYAVSPAYGSKFAKFSQMKLAFSKSAAVTSGVKAQFMDASGKVLREYNITAQSGNKTFTIGGIPQALNAGEEYTMKIPAGAFYLMADNSIKSDEITIKYIGRAEAPAAVQQVSPADQANVSEISSEHPVQILFDLSIAISEDAKAYLYRDGQTSPVCELNFVQGAESTILLYPSLKRYLEKDEKYKVVVEAGSVTDIMGFCPNNEITINYTGAYEPEISSDGSLFSDDFNDPSNSMVKYLLYEGDHNKPSSAMQDLGFDADNSPWLFVIRESESSSDYCAASTSIYNPTGKSDDWMAIPRLSIENADYYLSFDVQSYYKSKADRLKVLVLEDDAVYSNFTTELYEKFKANGKVLYDEQLSPGESEENLTGDWTHVEKSLAEYAGKNIYIAFVNENENQSMIFLDNLKVYYKGDFNFVPNVESTQVNKESTNVGVIVKVTSDKTYNTINATLTSEDGSFKSTYTDTPSKPITSAENYSFTFPDKLPLTVGAQNKYTISIDLGGTVYSQTNTISNLAFETTKHVVIEESTGQQCKNCPQGILAMENLEKLYGEQVIPIAIHSSIIGTDQFAYENYNTYFGITAQPMGLVNRIDTLYAPMYVDGSEQYHFDSPEGNNTFYDVAQREFENYAIADVSIDKAIYDASSKNIQITGNVNYALTMNSLNHNLAFVVLEDGLEGPQLNGFYVLDQPIFGEFGKGGKYGSSVAVVTFNDVARKVPNDNFAGESGFIPVSVTAGQPVAFNKVFSLPENVKNWDNTKVVVMLLDANTERVLNAARLKMSAGTAGINDATVSENGITISGENGSISVNGGSDLNVTVYDVSGSVISNVNSTSGAVKVSTGGKNGLFIVKATSDGVSVVKKVIVK

SEQ ID NO: 13 - DNA, 3729 bp, Prevotella rara
ttgggcctgctgtgggcaattccgtcttcagcacaggaagcacagcttaccactgtgagtttccccaaggctgcagctttcacatctttgtcagacaatggcttgtgggctactgctgctggtgtgaatgatgatgatcaaagtaagtatgcctatccttatcttattaatgtagagacaggtgctcttactgaactttgggttgaagcagacttgataaagtcactcgaagcaacagacgttactaatgatggaaaaatcatcgttggtacctatgacagcaagcctgcttattatgacatgaatcagggtaagtggatcactcttcagtctgagaatcctggaaaagctacatctgtaacacctgatggcaaatacatcagcggatggagcaattctggtagcttctcaggtgatgcttatgttgaaacaccgcttttgtgggagaagcagtctgatggtacatatcgtgcaattgatgtgtatgctgaacttcctaacttcccaaagaaaacaaagcttggaacaaacactcagcaggtacgtatagacaatgttagtcctgatggtaacatcctttctggtattattaactttgtaactcctgcaactgtttgctattatgtttacaacaagacaactcaggagtgcaaatatgtagacaatgctctcggagaagtgcctgacgaaacatttgttgacgagtcaacaatgagtaacaatggtaaatatcttaccggtatcgtacaggtggctggtggttcatacatttcaagctatctttacaatacaagtgacaactcttgtatattatataatacagaaagcgaagagcaagaccgtgccggaagtgctgtttcaaatacaggcgttgtatttgcttgcagtcctgccgtaaaccctgtccgttctgcttacgtacgtgtgggtagtctttggtacggaatagacgaaattctttctggccgttatgatatgaacttctatgagcgtactggctatgatttcacaggaacaattcaaggagtttctgatgatgaaaagaccataatcggtatgtctgaaacaaagacaaagggttatatcattcgtcttcctgaaactatcagcgaagctgcaagcagcgtgaatccattaggcacttatgccgtttctcctgcttatggctctaagtttgctaaattcagtcagatgaagttggctttctctaagtctgccgctgtaacatctggtgttaaggctcagttcatggacgcttctggtaaggtgttgagagagtataacattacggctcagtctggtaacaagacattcactattggcggtatacctcaggctctgaatgcaggcgaggaatatacaatgaagattcctgctggagcattctatttgatggcagacaactctatcaagagtgatgaaatcacaattaagtatatcggccgtgccgaggctccggctgctgtacagcaggtttctcctgcagatcaggcaaatgtatctgaaataagttcagagcatcctgtacagattctcttcgatttgtctatcgctatatctgaagatgctaaggcttatctgtatagagatggtcagacatcaccggtttgtgaacttaactttgtgcagggagcagaaagcacaatccttctgtatcctagcctcaagcgttatcttgaaaaagatgagaaatataaggttgttgtagaggctggttctgttacagatattatgggattctgtccgaacaatgagattacaattaattacacaggtgcatacgagcctgaaatcagttctgacggaagcctcttctctgatgacttcaatgatcctagcaactctatggttaaatacctcctttatgaaggtgaccacaacaagccgtcaagtgcaatgcaggatttaggctttgatgccgacaattctccttggcttttcgtaatccgtgaatcagaaagcagctctgactattgtgcagcttcaacatctatctataatcctacaggaaaatctgacgactggatggcaataccccgtctgtcaatagaaaatgccgactattatctcagctttgacgttcagtcatactataagtcaaaggcagacagacttaaggttctcgttcttgaggatgatgctgtttattctaacttcacaacagaactttatgagaagttcaaggctaatggtaaggttctttatgacgagcagctttctcccggtgagtcagaggaaaatctgacaggtgactggacacatgttgagaaatctctcgcagaatatgcaggtaagaatatctatatcgctttcgttaatgagaacgaaaatcagagtatgatcttcttggataatctgaaggtttactacaagggcgacttcaacttcgttcctaatgtagaaagcacgcaggttaacaaagagtctacaaatgttggtgtaatagttaaggttacaagtgataagacttataacactattaatgcaacacttacttctgaagacggctcattcaagagcacttatacagatacacctagcaagcctataacaagtgcagagaattattctttcacattccctgacaagttgcctctgactgtaggtgcacagaataagtatactataagcattgatctcggcggtactgtttacagccagacaaacactatcagcaaccttgcttttgagacaacaaagcatgtagttatagaagaaagcactggtcagcagtgtaagaactgtcctcagggaatccttgcaatggaaaatcttgagaaactttacggtgagcaggttatacctatcgctattcatagctctataatcggaacagaccagtttgcttatgagaactataatacatatttcggtataacagcacagcctatgggtctggttaatcgtatagacactctttatgcgccgatgtatgttgatggaagcgagcagtatcacttcgattcaccagaaggcaacaatacattctatgatgtagctcagcgtgagttcgaaaactatgcaattgcagatgtcagcatcgacaaggctatttacgatgcttcaagcaagaacatacagattacaggtaatgtaaactatgctctaaccatgaactctctgaaccacaatcttgcatttgttgttcttgaggatggtttggaaggacctcagcttaatggtttctacgttctcgaccagccgatattcggtgagttcggtaagggcggcaagtatggttcaagcgttgctgttgtaacattcaacgatgttgcacgtaaagtgccaaacgacaacttcgcaggtgaatcaggtttcatccctgtaagcgtaactgcaggtcagcctgttgcattcaataaggtattcagcttgcctgaaaacgttaagaactgggataacactaaggttgttgttatgttgctcgatgcaaatacagagcgcgttctgaatgctgcaagacttaagatgtcagccggaacagctggaatcaacgatgcaacagtatctgaaaacggtatcacaatttctggtgagaacggttcaataagcgttaacggcggaagcgatctcaacgttacagtttatgatgtaagcggaagcgtaataagcaatgtcaactctacttctggtgctgttaaggtaagcacaggcggaaagaacggcttgtttatcgttaaggctacaagcgacggcgtaagcgttgttaagaaagtaatcgttaaataa

SEQ ID NO: 14 - protein, 1230 aa, Prevotella rodentium
MRKNKLKTFLLAVIGISSFACVTLHAQNVTEPKMTLYDFKDQSMIYSLSDNGQWAVSYGTSPTDASRYTNARRTNVKTKESDILGLDGDETIPLQCQANDVADDGTVVGAYHDQPAIWTKAGGWKYLPIPKGWTTGFASAVTPDGHYAVGRMFSYSGNAENYGEYPMLWDLTTMQITETPGYPTVGSAGEKARMIRYDAISSDSRYITGIVDFSYTWNTLHFIYDRQNESYTTMGFNTDGTPWTEGLLGVEGTLSPNGKWFGGTAFIQNATNPNDEYSVPCRYNMETNEFEMFNELEARDYGSITIDNTGTIYSATPSSTPIRSVYIRAGKFWYALDELMSQSYGIDFYGKTGLDNTGTIMSVSADGKVITAFPDPYKSYILELDETLTDAAGRVNLLNNYTVTPANGASFSQMKDVSIKFSRDIKILGKTSDIKFTDDSGASVGRIITFAVSPSSSKTARIAFRTLNLTAGKKYTLTIPAGTIALSADETRLNDEIVITYTGRGTEPVKVVTAVPESGSALSQLNVTTNPILLTFDTNISLTENAAATLYRDGSDDIVSPLSVAVKDNQMLIYPETTQYLYLNTNYKVVLNAGSVTDVNGGNANERYEIMYEGIYERIVVADDTLIYKEDFANGVGGMMLYDGDGNIPNEEMKDYDFYYNNTPQPWVPVRESRESDDYSAASTSAYSPAGKSDDWMVTPQIYIPDAKCRLEFNGQGFRKYKQDKLKVIVYASDKVLNYFSKDNADEFRADGNVIMDEILSPGNSEDNLSNEWTTYSFKLDKYAGKNIYVAFINENEDQSIVFVDNIKVVRDNGFLTALTSATTVVGQNSHKIEGRVTANSETETYTTANIKLLDSEKNVVDEISENGLSLKKGDRYDFAFAKNLPLTIGEINVFYIRVQLDEKFDTISYAIKDLAFQPTKRVIVEEMTGQDCGNCPRGHLAWENLERVYGDRVILAGYHVYTGDIYESGMSSYVNQFLGLAGAPSAKVQRGETIGSPTYASITAGRTSYSFTSPLGDCWFDLVQKEFDTDADANLDVIAYFDEATQKVKATASAKFAMNISKQNIGLFIIVTEDGLPGFQHNYHYNDDADGLGEWGKGGTLGQEYVVYTHNDVARAQVGSYYGTTGYIPSTIASNETYTANIEFAKPAVNEIYNSNVICMMINANTGAVINVAKSKIAKASGIEGITTSGTDATEKIRYNAAGQIITAPVKGLNIIRMGDGSIRKVVVK

SEQ ID NO: 15 - DNA, 3084 bp, Prevotella rodentium
atgttttcatttatgggcatcggacaggccatagccgatgttgtgggttcgggatcaaaagaagatccgtacgtgcttgaaaacggcacaacactgacattgaaagcataccagtctttctatgccaaattcacggccccggctgacgggatcttctcattatatacaaaagacagctatgccctatataccgacgagagtttcagtcagattgacgagtcggcaaacattacattcaacggaagctacagtgagacggcatactactttaactgtaaagcaggtgttacctattatataggaaacagttttgtaatggtcggaggtacggttacagccaaattcaacacagaggctgaaccattggttctgcgtgaaatatcacctgaggccggttctgttttcaatgcaggcaaaggaagcgtagaactgacattcaaccaaaaagtccaaatagcttctgttactgtcaatgctggcacatcctcaaagacaatgtcagccaatgtaaatggagtatatgtatctgtagacgtaaaagactggctgaaccaaatgtatgatgaaggtaaggtcaaagaaggaaatgagatcagcttcaagttcaaaggcgtggccccaaccatttctccaagcaaattatacaacggcaatggagagttggacattacatacacagcaggcaagaaacccctgcaacttgtaagcagtaccaacaccccaatgagcactcctgccgtaaccacattcaagtcattctatacatccgatgacaaccaaggcatcgtaacactggaattcagtgacgaagtgaacttttcggaaggcaacaaaccaaccgcaacccttacatatggaaatatggaccaagatgccgacggcgaatactacacagaatcactccccatacttccacttggaagcaacattttaatggttaatctcaaggacaagctgcgccgtgcacaggacatggtgacttccggcactgtttacgacggaataacactatccatatcacacgtaaaggatatggacggaaactatgcctatggctcgggctccggtgtactcggatcgttcgcattcaactacaaactatctgaaataaactataccgttgatacagactgggcactacttgacgcaaccggcaatccgacaaacaaagacgtcatagattcagacaccaaaagcatagaactatggatgagcgaaaacgacggtcagataacattcaacggagtagaattcaaatataccgaaagcggtactgaaaaggtcaagacaatgaccctcagcgagattaaagttgacaacaatggaaacgaaacaacaataacaatccccgttcccaacatcgcagccgatgccggtagcgacatcgccatatctctcaaagacgtggaacgccccgacggtattaccaccagtatcgatccggccgcactaagctatttcacaaaaacattcacaacaacaggcataactgaaagcaaattcgacattacaagtgccatatggatgtatgaagagaatgaaggcaatattgtcgaagtcaatatgataaacggtaatatcggtgtactgacaagaggcagcaaatctgtaatcaaaaccaacaaagacaatgagattggttatgtagaatgggaaatcagaggcgttgacaatcctgatatggaatatatcagagctggatatgtagatacaaccatgacaggcaagttggtagacggctttaccatagaatggagaggagaaggcttgacagccggcaaagactacactttcacgcttcaggcatggaagaatgaagccgacaaaaacagtggtgccgagcctaatgtaggtgaagcaatgttcatcatacacggtacaaaacaagcctacatttacagcgatgttgtgatgaagactgatataagccagcctatcagacttgcttctgccaatgacaattaccgtaccatcgagttcagcgctcctgtaacgttaaatgccgtggtaaaccttggcatggggacatcggcagattgcaccgttgaaccctcggccgaccgtactgcatggacagtcacaatacctgaatatgtaatgtcacaatatggagagttcagcgtgaatgtctttgcaaaagatgacgaagggcgtgcagtaaacaagactgagaacggactgggtataataatggggacagaagacaatacgtggttccagattgattttgtcagtgagagccttgccccggactttacagtaacaccggcaaacgaatcagtgctcgagagtctcagcaccgtcactttcggttatgaaggcagtatcagcatcaactggaacaacagtgagaaaatcaccatatataacagaacaacacgtgagaagatagcagagttcagcggtgatgacgtcgtgttggatgaagatccggatgactattgggctccaatactctcatgccacatcacacttcccgagcctgtcactgctattggagtctacgatgtaaatgttcctgccggtttcttcgttcttggtgagcagttcgacagtaacttaagtaaggcaacaagcatagtatacgaaataaaggaaccggttgagccgttcggaatagaaataagccctactgccggattggtaagcgagattccgtcaaaactcatagtaacggtaacggacagaagcagttgtaactttactgccaaccccacattgaccgacaataccggtaacagctatcccgtacacaacgatttcgactggggtatcccggaaatgaacaagttcgtcatcattcttgacaacggagccatcacggctgacggaatatacacactcactattcctgccggctcgattataggtgacgacgagacagacctcaacaaggaagactttgtattcatatatacaatcaatctggccggaatcacagaactcgtcaacaatgagggcggaaaggttgacgtatacactctcaaaggaacattgttgatgaaagacgccgatgcatcagcagtaaacaagctggcaaaaggcatgtacataatcaatggtaaaaaagtgttcataagataa

SEQ ID NO: 16 - protein, 1212 aa, Prevotella muris
MKKTIALFVWSFIFILGLSAQSESPVLKTLEIPFGTICGMSDNGRWAVYDDGNDGVERGCSVDVYDLATGTIVTLSEGTEGDNIHLNDISDDGKIVAGSYNNVPAYFKDGKWTVLPLPAGTRGYGGRVSSMTPDGSVMVGMIYNNSFNFTSCYWKDGNLITLEGLPTTDISGKENAELNIVAVSADGNIVLGGLSTNHPGWGCCYFVYDVRTKTYEMLGQNLTSESFIDNVVMSNNGSFVGGNAYIVREVEGSEWPEELIVPFLYDVNKKTFEIYESTADNDQFVSAVANDGLMFCATPYGNPVRTMSVRVDGKYIDLGMILKQRYSIDFTKAMGVEYTGTAVAVSDDGKTIVAFPSPQDDNYALTLPVSFSEAAQGVNILAEYELSPVSGSSIAKIRQVALSFTREATVAEGAEAYIYKGETKLAVTNSISAASVKDNRIFILDFPETAFSEDEEYVLKIPAGIFVNGNMRNNEITAVYKGRADRPVAPTRIAPLEGSVITELSYNNPVMITFDTKIAVAQAVTGILFQSGSEQPLSSLVLVADGNKLYVYPPTTRRLMKGSDYVVKIPAGAVSDIVGFCPSNEITVNYHGAFVVTPPEQGSSFLFVDDFNDPGTSLSKWLMYEGDHNTPTSEMVGWGFDADNTPWNFSVHDNGQYDYCAASTSMYSPAGKANDWMITPQLSIGNEYYRLNFQTQSYKAGKTDKLKVYVWENNELIEGTVLKEHIDAIRANGKLVFDGILTPGANEATLTGEWESHSISLAEYAGKKVYIAFLNENEDQSVVFVDNVNVIYKGNFVAGSMTQENVVSQEEVEIKGYVMVTNNISYDAIEATYKTVDGTQIGIYKAEGIGLKEGSVYEFTFPEKLKLTKGQETQFTIVVKMGTEEQEINASVKNLAFNPKRRVVLEEGTGAWCGNCPGGILAVEYIESQFPGQLIPVCIHNDDAYAYGAYENFLGFRSFPTGRVNRIENYLSYMDSDEEGNPSFFSVDGDVTFADYVKSEIDKLTDVEIETGEAVYNSSTDEITVPVDVRFALDKNSVNYNILTVVVEDNLYANQRNYFASRTDPIYGDWGLGGKYGRGSVWYAYKDVARAIVGQSYYGENGYIPTSVRGGETITGNVSFEVPGKSITSLQNCKIVCMLIDAANGYVLNAARCDAISNALEWDLANGIEDAVVDTDTAGVENYNLAGQKMNAQRKGLNIVRLSNGRTVKVVK

SEQ ID NO: 17 - DNA, 3639 bp, Prevotella muris
atgaaaaaaactattgcattatttgtatggagtttcattttcatattagggctttccgcccaaagtgaatctcctgtattgaaaactcttgaaattccattcggtactatttgcgggatgtcagacaacggccgttgggctgtttatgacgatggcaatgacggtgttgagcggggctgttctgtggatgtctatgacttggctacaggaaccattgtaacactctctgaaggaacggaaggggataatattcatttgaatgatatttcggatgacggtaagatagtggcaggttcatacaacaatgttcccgcttactttaaggatggaaagtggacggtacttcctttaccggccggcacacgtggatatggcggaagagtttcgagtatgactccggatggttcggtaatggtcggaatgatttataataactcctttaattttacgtcatgctattggaaagacggaaatcttatcactcttgaaggattgcctacaaccgatatatccggtaaggaaaatgcagaattgaatattgttgctgtttcggctgacggcaatattgttctcggaggattgtcaaccaatcatccgggatggggatgctgttattttgtatatgatgtcaggacaaagacttacgagatgcttggtcagaatcttacctcagagtcattcattgataatgttgtgatgagcaataacggaagttttgtgggtggtaatgcatatatagtgcgtgaggttgaaggttcggaatggccggaggagcttattgttcctttcctttatgatgtgaataaaaaaacgtttgaaatatatgaaagtacagctgataatgaccagtttgtttcagctgtggcaaatgacggtttgatgttctgtgccactccgtacggtaatcctgtgcgtacgatgagtgtgcgtgtggatggaaaatatattgatttgggaatgatactcaaacaacgctattcgatagattttacaaaggcaatgggtgttgagtatacgggaactgccgtagcggtgagtgacgatggtaagacaatagtggctttcccttctccacaagatgataattatgccttgactctccctgtttcattctctgaggccgcacaaggtgttaatattcttgcggaatatgagctttctcctgtgtcaggaagcagtatcgcaaaaataaggcaggtcgctttatcttttacgcgtgaggccaccgtagctgaaggtgccgaggcatatatttataaaggtgaaacaaagttggcagtcacaaattccataagtgcggcgtctgtaaaagataatcgtatatttatacttgattttcctgagacagccttttcggaagatgaagagtatgtgcttaagatacctgcaggtattttcgtaaatggaaatatgagaaataatgaaatcacggctgtatataaaggacgtgcagacagaccggtagctccaacacgcatagctccgttggaaggaagcgtaataacagagttaagctacaacaatcctgtcatgattactttcgacacgaagattgctgtggctcaggcagtcacaggcattcttttccagagtggttcggaacagccgttgagcagtcttgtacttgttgccgatggaaacaaactatacgtatatcctcctacaacgcgtcgtttgatgaaaggttccgactatgtggtgaagatacctgccggtgctgtttccgatatagtagggttctgccccagtaatgagattactgtcaattatcatggggcttttgttgtaacacctcccgagcagggttcaagcttcctgtttgttgatgacttcaatgatccgggaacgtcactgagcaaatggcttatgtacgagggtgaccataacacaccgacctcagaaatggtaggatggggatttgatgcagacaatacgccatggaatttctctgtgcatgacaacggacagtatgattattgtgccgcatctacttccatgtattctccggccggcaaggcaaacgactggatgataaccccacagctttctataggaaacgaatattacagactgaatttccagacgcagtcatataaggccggtaagactgataaactgaaagtttatgtatgggagaacaatgagcttatagaaggtactgtgctgaaagagcacattgatgcaatacgtgcaaacggaaagctggtatttgacggtatactgactccgggagcaaatgaagctacgcttaccggtgaatgggaaagccacagcatttcacttgcagaatatgcaggaaagaaagtgtatatagcattcctcaacgaaaacgaagaccaaagtgtagtgtttgttgataacgtaaatgtaatatacaaaggcaactttgttgccggaagcatgacacaggagaatgtcgtctcacaggaagaggtggaaatcaagggatatgtaatggtgaccaacaacatatcatacgatgccattgaggccacatataagacggtagacggaacccaaataggaatttataaggctgagggtatcggtttgaaggagggcagtgtttatgaatttacgttccctgaaaaactgaagttgaccaaagggcaggaaacgcagtttactatagtggtgaagatgggtacggaagaacaggagataaatgcttcggttaagaatcttgcgttcaatcccaagcgtcgtgtcgtacttgaagaaggcaccggcgcatggtgtggaaattgtcctggaggtatacttgctgtggaatatattgaaagtcagttccccggtcagttgatacctgtatgcatacataatgacgatgcgtatgcttatggtgcgtatgagaatttccttggtttccgctcgttccctacaggtcgtgtaaaccgtattgagaattatctttcatatatggactcagatgaggaaggcaatccgtctttcttctctgttgacggagatgtaacgtttgctgactatgtgaagagtgagatagacaaacttacagatgttgaaatagagacaggcgaggctgtctataattcgtctacggatgagataactgtgccggtcgatgtaaggtttgcccttgacaagaattctgtaaattataatattcttactgttgttgtcgaggataatctatatgctaatcagcgtaattattttgcaagccgtacggatcctatttatggagactgggggcttggcggtaagtatggccgtggttccgtatggtatgcttataaggatgtcgcacgtgcaatcgtgggtcagtcttattatggtgagaacggatatattcccacttctgtcagaggcggtgagacaataactggtaatgtttcttttgaagttcccggcaaatcgattacttcactgcagaattgcaagattgtatgtatgctgattgatgcggctaacggatacgttcttaatgcagcacggtgtgatgcaatatctaacgcattggaatgggatcttgcgaatggaatagaggatgctgttgttgatacagatacagcaggtgtggagaattacaatctggcaggccagaaaatgaatgctcagcgcaaaggtcttaatatcgtaaggctttccaacggacgtacggtgaaagtcgtaaagtga

SEQ ID NO: 18 - protein, 1027 aa, Paraprevotella clara
MREKLYTKWKGGLNRLCFLLMCFCWTTVQSWAVGEDLHLTIENGKTYEFEAFNSYYLTYVATANGQLSLYQTGGDFCRQYTDNTFETELPSTPQYVNEGKLVEVKVESGKTYYFLTRGLSKGELTVTFGEKATPLELLSLSKEEGTTLNLSIDTLLGFTFNRMVKVGNCTLSSGSVIGNLTASTHDYGFTVSIKDVLYKWLKEGNVKAGDEVVLTVTGLCNANDESDKYNGNGVLTVKYIAGALPAELVSVANSPEEMNFLSYYLPTDERGLVTLTFNRSMGEDATAKLFYGDIEGSNVYTESLPVKVKDTQLIVDLRGKRRLPSDMLPNASADVWEQYKTISLKVSNVRDAEGNYAMSTSQGTTGSYAFNYTIEAVEFDIARQFTPDEGTSLDDYPTIELWIREDDSFTYEGVDFTYSVNGKPETVFVPISQITKKDSPDGDGVLLTIPVPNKAADENSDVVVSLNNLKAADGADYSEDFTIIYKTSGKSMAGLEIESVSPADGAAIAALEAGSFLELSTNMNDRVGYVWFRIDDQNPKDPDQACVKTMTSMKKETVEGKVSFRTEIIRSVTFFEGHTYKVTFNAYASESDYQHGADALGVMTVTYTGTTPEFKFSPVKFVGITPDPDYTVISDVSQNEFTLTFDGPVVLNHENAFVVYGQGMNYPFESIESNEDGTEWTVKASLEKLMEMGMMPRLSMSFMPVDKDGMLVEGNAGKDATSYLNFAYDCTIGIPDLQVSPESGSKVESLKEIIVGCKDIMDDNGEVIFQGGISESYMAAEKIILYKNGREPVATVTSIEPIIPEDQEDNYFYVPVEMKLTLDTEITDNGNYRLHIPANYFILGTGMSNVNSKETSVLYTIDQPIKITVTPENNSTVESLKEITIECESGIDVPSMGTIQLLNAQNEVVASATGEDCELLLPEGAGPWDPYTGVTIKLDQEVTEKGTYKLVIPEGFFYLGENYENSDEMTFTYSINASGIHSIGTESKGVVVYTVDGKFILKSSDAKDVKNLKKGLYIVNGKKMMVK

SEQ ID NO: 19 - protein, 1027 aa, Paraprevotella clara
MREKPYTKWKGGLNRLCFLLMCFCWTTVQSWAVGEDVHLTIENGKTYEFEAFNSYYLTYVATANGQLSLYQTGGDFCRQYTDNTFETELPSTPQYVNEGKLVEVKVESGKTYYFLTRGLSKGELTVTFGEKATPLELLSLSKEEGTTLNLSIDTLLGFTFNRMVKVGNCTLSSGSVIGNLTASTHDYGFTVSIKDVLYKWLKEGNVKAGDEVVLTVTGLCNANDENDKYNGNGVLTVKYIAGALPAELVSVTNSPEDMNFLSYYLPTDERGLVTLTFNRSMGEDATAKLFYGDIEGSNVYTESLPVKVKDTQLIVDLRGKRRLPSDMLPNASADVWEQYKTISLKVSNVKDVEGNYAMSTSQGTTGSYAFNYTIEAVEFDIARQFTPDEGTSLDDYPTIELWIREDDSFTYEGVDFTYSVNGKPETVFVPISQITKKDSPDGDGVLLTIPVPNKAADENSDVVVSLNNLKAADGADYSEDFTIIYKTSGKSMAGLEIESVSPADGAAIAALEAGSFLELSTNMNDRVGYVWFRIDDQNPKDPDQACVKTMTSMKKETVEGKVSFRTEIIRSVTFFEGHTYKVTFNAYASESDYQHGADALGVMTVTYTGTTPEFKFSPVKFVGITPDPDYTVISDVSQNEFTLTFDGPVVLNHENAFVVYGQGMNYPFESIESNEDGTEWTVKASLEKLMEMGMMPRLSMSFMPVDKDGMLVEGNAGKDATSYLNFAYDCTIGIPDLQVSPESGSKVESLKEIIVGCKDIMDDNGEVIFQGGISESYMAAEKIILYKNGREPVATVTSIEPIIPEDQEDNYFYVPVEMKLTLDTEITDNGNYRLHIPANYFILGTGMSNVNSKETSVLYTIDQPIKITVTPENNSTVESLKEITIECESGIDVPSMGTIQLLNAQNEVVASATGEDCELLLPEGAGPWDPYTGVTIKLDQEVTEKGTYKLVIPEGFFYLGENYENSDEMTFTYSINASGIHSIGTESKGVVVYTVDGKFILKSSDAKDVKNLKKGLYIVNGKKMMVK

SEQ ID NO: 20 - DNA, 3084 bp, Paraprevotella clara
atgagagagaaaccttacacgaaatggaagggaggcctgaataggctttgttttcttcttatgtgtttttgttggactacggttcagtcatgggccgttggtgaagatgtacatttaaccattgaaaatggtaagacgtatgaatttgaagctttcaacagttattatcttacttatgtagccacggctaacggacaattatcattgtatcaaaccggtggagacttttgtcgtcagtatacagataacacttttgaaacggaattgccttctacccctcagtatgttaatgagggaaaacttgtagaagtgaaggttgagtcaggtaagacttattatttcttgactcgaggtttaagtaaaggagaactgaccgttactttcggagaaaaagcaactccacttgaattactttcgctctccaaggaagagggaacgacattgaatctttctattgataccctcttaggcttcactttcaatagaatggtaaaagtaggaaattgcacattgtcttccgggtcggtaatcggaaacttgaccgcttcgacgcatgattatggtttcaccgtttccattaaagatgtgttgtataaatggttgaaggagggtaatgtaaaagccggagatgaagtcgttttgactgtaacgggattatgtaatgccaatgatgagaacgacaaatacaatggtaatggcgtgctgacggtgaaatatattgcaggagcgttgcctgccgagttggttagcgttacgaactcacccgaagatatgaacttcctgtcttattacctgcctactgatgaaagggggttggttactttgactttcaaccgttcgatgggcgaagatgctacggcaaaattattctatggcgatatagaaggttcgaatgtctatacggaaagtcttccggtgaaggtgaaagatactcagttgattgtagacctccgtggaaaacgtcgtttgccatctgatatgttgccgaatgccagtgctgatgtttgggaacagtataaaaccatttccttgaaggttagcaacgtgaaggatgtggaaggaaattatgctatgtctacctctcagggtaccacaggttcgtatgcttttaattatacaatagaagctgttgagtttgatatcgctcgtcagtttacaccagatgaaggcacatctttggatgattatccgacaatagaactttggattcgggaagacgattcgtttacttatgagggtgtagatttcacttatagcgtgaatggaaaacctgagacggtatttgtacccatcagccagattacgaaaaaagactctccagacggagatggtgtactattgacgattccggtgccgaataaagcagcggatgagaattcagatgtcgtagtttctttgaataatttgaaagcggccgatggtgcggattattcagaagattttacgataatatataaaacgtcaggaaagagtatggcagggcttgagatagaatctgtgtctcctgctgatggagcagctatcgcggctttagaagctggttcgtttctggaattgtctaccaatatgaatgatcgtgtaggatatgtatggtttagaatagatgaccagaacccgaaggatcctgatcaggcttgtgttaagacgatgacatcgatgaagaaagagacggttgagggaaaagtttctttccggacagaaataattcgtagtgtgactttctttgaagggcatacttataaagttactttcaatgcttatgcttcggagagcgattatcagcacggtgcagatgctcttggtgttatgactgtgacttacacaggtacaactccggaatttaagtttagtccggttaagtttgtaggaataacgccggatcctgattatactgtaatttcagacgtaagccagaatgaatttacgttgacttttgacggtcctgtagtattgaatcatgaaaatgcttttgttgtatacggtcagggaatgaattatccatttgaaagtatcgagtcgaatgaagacggtacggaatggacggtaaaggcatccttggaaaaattaatggaaatgggtatgatgcctcgattgtctatgagctttatgccggtggataaagacggaatgttagttgaaggtaatgccggtaaagatgcgacaagttatttgaattttgcctatgattgtacgattggtataccagatttgcaagtgagtccggaaagcggttctaaagtggaaagtttgaaagagatcatagtaggatgtaaagatatcatggacgacaatggtgaggtgatatttcaaggtggtatcagcgaatcttatatggcggccgaaaagatcattttgtataagaacggacgtgagccggttgcaacggtaacgagtatcgaacctattataccggaggaccaagaggataattacttctacgttcctgtggaaatgaaattaacattggatactgaaattacagataacggtaattatcgtttgcacattcctgccaactactttatattgggaacaggtatgtctaatgtaaacagtaaagaaacaagtgtgctgtatactatcgaccagccgattaagataacggttacgccagagaataactctacggtagaaagcctgaaagaaattactatcgaatgtgaatcaggtatagatgtgccgagtatgggtacaattcaattattgaatgctcagaatgaggtggtagcttcggcaacgggtgaggattgcgaattgttgttacctgaaggtgccggtccttgggatccttatactggtgtgacaattaaattggatcaagaggtgacagagaaaggtacatataagttggttattcctgaaggattcttctatttgggtgaaaactatgaaaattcggacgagatgacgtttacttattcgattaatgccagtggtattcattcgattggtactgagtctaagggagtagtcgtttatactgtagacggtaaatttatcttaaagtcgagcgatgccaaagacgtgaagaatctgaagaaaggtttgtacattgtgaacggtaagaagatgatggtaaaataa

SEQ ID NO: 21 - protein, 787 aa, Paraprevotella xylaniphila
MRKMFTLEMKDYLMRMVLFVAVCMVGVGGLKAAPGLSADDPLIFEGGEEYDVSGSYFKDLYATFTAPSDGVLTLTFDSTDPLDLYTDNTYQTMVEPRLVYNNGVCELEVKAGITYYFHRSFMLSARTISVEFGKEAVALKLQRVSPTEGETLFVSNATVSFTFNRDVKMDGATLTIGGKEKSIDAVSTSSSVQFDLSAIMMEAYNDGILKEGDDMLLTLKGVRNANKESDIYGEDGTCSLALKAAAKPVVLNSSVNTPGNGMDIFHSYIMSGDENVVQLNFDGALDTEKKPVATLIYGDIEAENGFYQETLDAQFLGENTVTVDLSGKSRRHKDMLPNYSGAAFGTISLKIAGVYAADGQPVYSGAQSSVGSCTFQYAYEEVKVDIAVAFDDLAESNSIDGLDSLTIWVRGDEYLHYTGVQFDFMVNGQVNSIVEKDIKKKADSEEEGACILRVCVPKSDADANSEVKVSFVGLEAADGGDYSADFSAVFTTVGNLVNVPDLILTPVSGSTVENIKEVLVGCSEGIRVNADNKEKIQIWDRMRNVVATAVSMEPVIPEDEKENPDYIPTEIKVVFDNEVKLPGAYMVNLPAEAFVLGNQTSILSKATLVDYMIIGEVAKDYVPSEVVAETEGSTVIGFTIKTPEWVTLDENFDTEKIKIYNSNTQEEVVGGKSVSYAAAFEDFSIALENPLTEKGTYTLFIPAELFGNGSWIPGSTEGSCNPELTYTIVIDENGVTVGVNSVLAEIGTKVTVYNLNGVRVLYNADRDALKALRKGIYVVNGKKVVIK

SEQ ID NO: 22 - DNA, 2364 bp, Paraprevotella xylaniphila
atgaggaagatgtttactttggaaatgaaagactatctgatgaggatggttctttttgtggcagtgtgtatggtgggtgttggaggattgaaagctgcccccggattgtcagctgatgatcctttgatctttgaaggtggagaagaatatgatgtttcgggaagttattttaaagatttgtatgctacgtttacggctccttcggacggagtattgactttgacatttgatagtaccgatcctttggatttatatacggataatacatatcaaacgatggtggagccacgtcttgtttacaataatggggtttgcgaattggaagtaaaagccgggattacttattattttcaccgttcttttatgttgagcgcacgaaccatttctgtggaatttggaaaggaagctgttgctttgaagttacaacgagtttctccaacagagggtgagacattgtttgtttccaatgctacagtaagtttcactttcaatagggatgttaaaatggatggggctactcttacaattggaggaaaagaaaagtctattgatgcggtttcgacatcgtcttctgtacaatttgacctatctgccattatgatggaggcatacaatgatggaatcctaaaggaaggagatgatatgctcttaactttgaagggagtacggaatgcgaataaagaaagtgatatttatggagaagacgggacttgctccttggctttaaaagcagcagcaaaacctgtggttctaaacagttctgtaaatacgcctggaaatggaatggatatatttcattcttatattatgtctggggacgagaatgttgtacagttgaattttgatggtgctttggatacagagaagaaaccggttgcaacattaatatatggggatatagaagcggagaatggtttttatcaagaaaccttagatgcgcaattcttaggtgaaaatactgtaactgtagatttgagcggaaaatcgcgtcggcataaagatatgctgccgaactattccggcgctgcctttggaactatttctttgaaaattgcaggggtgtatgcagctgacggacaacctgtttattctggtgctcaatcctcagtaggttcttgtacgtttcaatatgcctatgaggaagtaaaggtggatatagctgtggcttttgatgacttggcagaaagtaattctattgacggattagactcattaacaatttgggttcgtggtgatgaatacttgcattacactggagtgcagtttgattttatggtaaatggtcaagttaattctattgtagagaaagatattaagaaaaaagcggattctgaagaagaaggtgcctgtatattaagagtatgtgtaccgaaaagtgatgccgatgccaattcggaggtaaaggtcagctttgttggccttgaagcagctgacggcggggattactccgcagatttttctgctgttttcacaacagtaggaaacttggtaaatgtaccggatttgatactcactccagtgagcggttctacagtggaaaatattaaagaggtattagttggttgttctgagggtattcgcgtgaatgcagacaacaaggagaaaatacagatatgggatagaatgcggaacgtagtagctacagcggtaagtatggagcctgttattcctgaagatgagaaggaaaatccggattacataccgacagaaataaaggtggtttttgataatgaagtgaagctccccggagcttatatggtgaatcttccggcagaggcattcgttttaggaaatcagacatctattttaagtaaggcaacccttgtggattatatgattataggggaagttgcgaaagattatgttccgagcgaagttgtagccgagacagaaggaagtacagtgataggttttacgataaagacaccagaatgggtgactttggatgagaattttgacacagagaaaatcaagatttataattcgaatactcaggaagaagttgtgggtggaaaatcggtaagttatgcagcagcttttgaagattttagtatcgcattggagaatcctctcacagagaaaggtacttatacgttgtttattccggcagaattgtttggaaatggttcttggattcccggttctacagaagggtcttgtaatccggaattaacttatacgatagttatagacgagaatggggtgacagtcggagtaaattcagtattggctgaaattgggacaaaagtaacggtgtacaatcttaatggtgtacgtgtgctttataatgcagaccgtgatgcattgaaggctttaagaaaaggaatttatgtcgtgaatggaaagaaggtggtgattaagtaa

SEQ ID NO: 23 - protein, 787 aa, Paraprevotella xylaniphila
MRKMFTLEMKDYLMRMVLFVAVCMVGVGGLKAAPGLSADDPLIFEGGEEYDVSGSYFKDLYATFTAPSDGVLTLTFDSTDPLDLYTDNTYQTMVEPRLVYNNGVCELEVKAGITYYFHRSFMLSARTISVEFGKEAVALKLQRVSPTEGETLFVSNATVSFTFNRDVKMDGATLTIGGKEKSIDAVSTSSSVQFDLSAIMMEAYNDGILKEGDDMLLTLKGVRNANKESDIYGEDGTCSLTLKAAAKPVVLNSSVNTPGNGMDIFHSYVMSGDENVVQLNFDGALDTEKKPVATLIYGDIEAENGFYQETLDAQFLGENTVTVDLSGKSRRHKDMLPNYSGAAFGTISLKIAGVYAADGQPVYSGAQSSVGSCTFQYAYEEVKVDIAVAFDDLAGSNSIDGLDSLTIWVRGDEYLHYTGVQFDFMVNGQVNSIVEKDIKKKADSEEEGACILRVCVPKSDADANSEVKVSFVGLEAADGGDYSADFSAVFTTVGNLVNVPDLILTPVSGSTVENIKEVLVGCSEGIRVNADNKEKIQIWDRMRNVVATAVSMEPVIPEDEKENPDYIPTEIKVVFDNEVKLPGAYMVNLPAEAFVLGNQTSILSKATLVDYMIIGEVAKDYVPSEVVAETEGSTVIGFTIKTPEWVTLDENFDTEKIKIYNSNTQEEVVGGKSVSYAAAFEDFSIALENPLTEKGTYTLFIPAELFGNGSWIPGSTEGACNPELTYTIVIDENGVTVGVNSVLAEIGTKVTVYNLNGVRVLYNADRDALKALRKGIYVVNGKKVVIK

SEQ ID NO: 24 - DNA, 2364 bp, Paraprevotella xylaniphila
atgaggaagatgtttactttggaaatgaaagactatctgatgaggatggttctttttgtggcagtgtgtatggtgggtgttggaggattgaaagctgcccccggattgtcagctgatgatcctttgatctttgaaggtggagaagaatatgatgtttcgggaagttattttaaagatttgtatgctacgtttacggctccttcggacggagtattgactttgacatttgatagtaccgatcctttggatttatatacggataatacatatcaaacgatggtggagccacgtcttgtttacaataatggggtttgcgaattggaagtaaaagccgggattacttattattttcaccgttcttttatgttgagcgcacgaaccatttctgtggaatttggaaaggaagctgttgctttgaagttacaacgagtttctccaacagagggtgagacattgtttgtttccaatgctacagtaagtttcactttcaatagggatgttaaaatggatggggctactcttacaattggaggaaaagaaaagtctattgatgcggtttcgacatcgtcttctgtacaatttgacctatctgccattatgatggaggcatacaatgatggaatcctaaaggaaggagatgatatgctcttaactttgaagggagtacggaatgcgaataaagaaagtgatatttatggagaagacgggacttgctccttgactttaaaagcagcagcaaaacctgtggttctaaacagttctgtaaatacgcctggaaatggaatggatatatttcattcttatgttatgtctggggacgagaatgttgtacagttgaattttgatggtgctttggatacagagaagaaaccggttgcaacattaatatatggggatatagaagcggagaatggtttttatcaagaaaccttagatgcgcaattcttaggtgaaaatactgtaactgtagatttgagcggaaaatcgcgtcggcataaagatatgctgccgaactattccggcgctgcctttggaactatttctttgaaaattgcaggggtgtatgcagctgacggacaacctgtttattctggtgctcaatcctcagtaggttcttgtacgtttcaatatgcctatgaggaagtaaaggtggatatagctgtggcttttgatgacttggcaggaagtaattctattgacggattagactcattaacaatttgggttcgtggtgatgaatacttgcattacactggagtgcagtttgattttatggtaaatggtcaagttaattctattgtagagaaagatattaagaaaaaagcggattctgaagaagaaggtgcctgtatattaagagtatgtgtaccgaaaagtgatgccgatgccaattcggaggtaaaggtcagctttgttggccttgaagcagctgacggcggggattactccgcagatttttctgctgttttcacaacagtaggaaacttggtaaatgtaccggatttgatactcactccagtgagcggttctacagtggaaaatattaaagaggtattagttggttgttctgagggtattcgcgtgaatgcagacaacaaggagaaaatacagatatgggatagaatgcggaacgtagtagctacagcggtaagtatggagcctgttattccggaagatgagaaggaaaatccggattacataccgacagaaataaaggtggtttttgataatgaagtgaagctccccggagcttatatggtgaatcttccggcagaggcattcgttttaggaaatcagacatctattttaagtaaggcaacccttgtggattatatgattataggggaagttgcgaaagattatgttccgagcgaagttgtagccgagacagaaggaagtacagtgataggttttacgataaagacaccagaatgggtgactttggatgagaattttgacacagagaaaatcaagatttataattcgaatactcaggaagaagttgtgggtggaaaatcggtaagttatgcagcagcttttgaagattttagtatcgcattggagaatcctctcacagagaaaggtacttatacgttgtttattccggcagaattgtttggaaatggttcttggattcccggttctacagaaggggcttgtaatccggaattaacttatacgatagttatagacgagaatggggtgacagtcggagtaaattcagtattggctgaaattgggacaaaagtaacggtgtacaatcttaatggtgtacgtgtgctttataatgcagaccgtgatgcattgaaggctttaagaaaaggaatttatgtcgtgaatggaaagaaggtggtgattaagtaa

SEQ ID NO: 25 - protein, 542 aa, Prevotella rara
MKRLIFTLIGIVLGLTGLKAVTFTPIEINDPSESVTIKLQPGANYLQLKAIESNTIHFNVGYFGIMMFECNAMGEEGNNLSISYDAEGHKIFSSEVEEGKTYYFSTSMITEPSIDVTIYYGNGEGMPITLTSNFSDGDTYTVSGSNLELAFDRTVDIAHNWIEYGEEADGVFKTKEEIPAAYINGTYTTQYFYSIELSKFIREMAEDGKLEVGDKFKITLEGICDANDESVIYGEDGNYSVTLIMGEMPGELVSIDSAQGTTLYTYYPETGEEGLLTFTFTDELNTDKSKVTVDLSYGDSEAGSMGSFNPDFTIEGKTVVVDIRGYRFPETVETSRNGEVQTVITMNIKGLTTADGRAILTNNASAGTSGIVVTYPLKKQEISFYYDFLPTEGSSLADCSEIIIWLPEEVGVLTFDKVLLQWLNNRGTLQTKEFKAEDVPFAYDKSYAGYVSHIPLAGVSKDREVTLTVEGGMLSNGDSVEITGKFNTDPTGIDSVLGDDANAVVKLYTIDGILVKEAPAATVLTGVKKGVYIMNGKKVVVK

SEQ ID NO: 26 - DNA, 1629 bp, Prevotella rara
atgaaacgacttatttttactttaatcggtattgtattggggttgacaggtttaaaggctgttacttttactccgattgagattaatgacccgtctgagtctgtaactattaaattgcagccaggtgcaaactatttacagctgaaggctattgagagcaacaccatccactttaatgtcggatattttggcattatgatgtttgaatgtaatgccatgggtgaagagggcaacaacctttctataagctatgacgctgaaggtcacaaaatcttcagtagtgaggttgaggaaggaaaaacttattatttctcaaccagtatgattactgagccttcaatagatgttacaatttattatggtaacggagaaggcatgcctatcacattgacatctaacttttcggatggtgatacctatacagtttctggctcaaaccttgaattggcttttgaccgtacggttgatatagcccacaactggattgagtatggtgaggaggctgacggcgtatttaaaacaaaggaagagattcccgcagcatatatcaatggtacctatactactcagtatttctatagcatcgagctgagcaagtttatccgtgagatggctgaagacggtaaacttgaggttggtgataagtttaaaatcactcttgaaggtatttgcgatgctaacgatgagagcgtaatctatggtgaggacggaaactattctgttacactgattatgggcgagatgcccggtgagctggtttctatagattcggcacaaggtacaactctttatacatattatcctgaaaccggtgaagaaggtttgctgacatttactttcacagatgaacttaatactgataagagtaaggtaactgtagacctgtcttatggcgattcagaggccggttctatgggttcatttaatcctgattttactatcgaaggcaagactgttgttgttgatatccgcggttaccgcttcccagagacagtagagacttcaagaaacggtgaagtgcagactgtgataacaatgaacatcaagggccttacaactgcagacggacgtgctattctcacaaacaacgcttctgccggaacaagtggcatcgttgttacttatcctctgaagaagcaggaaatatctttttattatgacttcttgcctactgaaggcagctctctggctgattgcagcgagatcataatctggttgccggaggaagttggtgttcttactttcgacaaggttctgttgcagtggctcaacaaccgcggcacactccagacaaaggaattcaaggcagaggatgttccgtttgcttatgataaatcttatgcgggttatgtaagccatattccacttgccggcgtaagcaaggaccgtgaggttacattgactgtagaaggtggaatgctcagcaatggcgacagcgttgagattacaggtaaattcaacactgatcctacaggtatagattctgttcttggtgacgatgccaatgccgttgttaagctttacacaatcgacggtatcctcgttaaggaggctcctgctgcaactgttcttacaggtgttaagaagggcgtttatatcatgaacggcaagaaggttgttgtaaaataa

SEQ ID NO: 27 - protein, 1027 aa, Prevotella rodentium
MFSFMGIGQAIADVVGSGSKEDPYVLENGTTLTLKAYQSFYAKFTAPADGIFSLYTKDSYALYTDESFSQIDESANITFNGSYSETAYYFNCKAGVTYYIGNSFVMVGGTVTAKFNTEAEPLVLREISPEAGSVFNAGKGSVELTFNQKVQIASVTVNAGTSSKTMSANVNGVYVSVDVKDWLNQMYDEGKVKEGNEISFKFKGVAPTISPSKLYNGNGELDITYTAGKKPLQLVSSTNTPMSTPAVTTFKSFYTSDDNQGIVTLEFSDEVNFSEGNKPTATLTYGNMDQDADGEYYTESLPILPLGSNILMVNLKDKLRRAQDMVTSGTVYDGITLSISHVKDMDGNYAYGSGSGVLGSFAFNYKLSEINYTVDTDWALLDATGNPTNKDVIDSDTKSIELWMSENDGQITFNGVEFKYTESGTEKVKTMTLSEIKVDNNGNETTITIPVPNIAADAGSDIAISLKDVERPDGITTSIDPAALSYFTKTFTTTGITESKFDITSAIWMYEENEGNIVEVNMINGNIGVLTRGSKSVIKTNKDNEIGYVEWEIRGVDNPDMEYIRAGYVDTTMTGKLVDGFTIEWRGEGLTAGKDYTFTLQAWKNEADKNSGAEPNVGEAMFIIHGTKQAYIYSDVVMKTDISQPIRLASANDNYRTIEFSAPVTLNAVVNLGMGTSADCTVEPSADRTAWTVTIPEYVMSQYGEFSVNVFAKDDEGRAVNKTENGLGIIMGTEDNTWFQIDFVSESLAPDFTVTPANESVLESLSTVTFGYEGSISINWNNSEKITIYNRTTREKIAEFSGDDVVLDEDPDDYWAPILSCHITLPEPVTAIGVYDVNVPAGFFVLGEQFDSNLSKATSIVYEIKEPVEPFGIEISPTAGLVSEIPSKLIVTVTDRSSCNFTANPTLTDNTGNSYPVHNDFDWGIPEMNKFVIILDNGAITADGIYTLTIPAGSIIGDDETDLNKEDFVFIYTINLAGITELVNNEGGKVDVYTLKGTLLMKDADASAVNKLAKGMYIINGKKVFIR

SEQ ID NO: 28 - DNA, 3084 bp, Prevotella rodentium; identical to SEQ ID NO: 15

SEQ ID NO: 29 - DNA, 1528 bp, Paraprevotella clara
atgaagagtttgatcctggctcaggatgaacgctagctacaggcttaacacatgcaagtcgaggggcagcatggactcagctttgctgagtttgatggcgaccggcgcacgggtgagtaacgcgtatccaacctgccctttactccgggatagtctcctgaaagggagtttaataccggatgtgtttgtttttccgcatgggagcgacaaataaagattaattggtaaaggatggggatgcgtcccattagcttgttggcggggtaacggcccaccaaggcgacgatgggtaggggttctgagaggaaggtcccccacattggaactgagacacggtccaaactcctacgggaggcagcagtgaggaatattggtcaatgggcgggagcctgaaccagccaagtagcgtgaaggacgacggccctacgggttgtaaacttcttttataagggaataaagttcgccacgcgtggtgttttgtatgtaccttatgaataagcatcggctaattccgtgccagcagccgcggtaatacggaagatgcgagcgttatccggatttattgggtttaaagggagcgtaggcgggcttttaagtcagcggtcaaatgccacggctcaaccgtggccagccgttgaaactgtaagccttgagtctgcacagggcacatggaattcgtggtgtagcggtgaaatgcttagatatcacgaagaactccgatcgcgaaggcattgtgccggggcagcactgacgctgaggctcgaaagtgcgggtatcaaacaggattagataccctggtagtccgcacggtaaacgatgaatgctcgctatgggcgatatattgtccgtggccaagcgaaagcgttaagcattccacctggggagtacgccggcaacggtgaaactcaaaggaattgacgggggcccgcacaagcggaggaacatgtggtttaattcgatgatacgcgaggaaccttacccgggcttgaattgcaggtgcatgagtcagagacggctctttccttcgggactcctgtgaaggtgctgcatggttgtcgtcagctcgtgccgtgaggtgtcggcttaagtgccataacgagcgcaacccttctccccagttgccatcgggtaatgccgggccctctggggacactgccatcgtaagatgcgaggaaggtggggatgacgtcaaatcagcacggcccttacgtccggggctacacacgtgttacaatggggggtacagagggccgctgtccggtgacggtcggccaatccctaaaacccctctcagttcggactggagtctgcaacccgactccacgaagctggattcgctagtaatcgcgcatcagccatggcgcggtgaatacgttcccgggccttgtacacaccgcccgtcaagccatgaaagccgggggtgcctgaagtccgtgaccgcgagggtcggcctagggtaaaactggtgattggggctaagtcgtaacaaggtagccgtaccggaaggtgcggctggaacacctccttt

SEQ ID NO: 30 - DNA, 1481 bp, Paraprevotella xylaniphila
gatgaacgctagctacaggcttaacacatgcaagtcgaggggcagcatgaacttagcttgctaagtttgatggcgaccggcgcacgggtgagtaacgcgtatccaacctgccctttacgcggggatagccttctgaaaggaagtttaatacccgatgaattcgtttagtcgcatggcttgatgaataaagatttatcagtaaaggatggggatgcgtcccattagcttgttggcggggtaacggcccaccaaggcgacgatgggtaggggttctgagaggaaggtcccccacattggaactgagacacggtccaaactcctacgggaggcagcagtgaggaatattggtcaatgggcgcgagcctgaaccagccaagtagcgtggaggacgacggccctacgggttgtaaactccttttataaggggataaagttggccatgtatggccatttgcaggtaccttatgaataagcatcggctaattccgtgccagcagccgcggtaatacggaagatgcgagcgttatccggatttattgggtttaaagggagcgtaggcgggcagtcaagtcagcggtcaaatggcgcggctcaaccgcgttccgccgttgaaactggcagccttgagtatgcacagggtacatggaattcgtggtgtagcggtgaaatgcttagatatcacgaggaactccgatcgcgcaggcattgtaccggggcattactgacgctgaggctcgaaggtgcgggtatcaaacaggattagataccctggtagtccgcacagtaaacgatgaatgcccgctgtcggcgacatagtgtcggcggccaagcgaaagcgttaagcattccacctggggagtacgccggcaacggtgaaactcaaaggaattgacgggggcccgcacaagcggaggaacatgtggtttaattcgatgatacgcgaggaaccttacccgggcttgaatcgcaggtgcatgggccggagacggccctttccttcgggactcctgcgaaggtgctgcatggttgtcgtcagctcgtgccgtgaggtgtcggcttaagtgccataacgagcgcaacccccctccccagttgccatcgggtaatgccgggcactttggggacactgccaccgcaaggtgcgaggaaggtggggatgacgtcaaatcagcacggcccttacgtccggggcgacacacgtgttacaatggggggtacagagggccgctgcccggtgacggttggccaatccctaaagcccctctcagttcggactggagtctgcaacccgactccacgaagctggattcgctagtaatcgcgcatcagccatggcgcggtgaatacgttcccgggccttgtacacaccgcccgtcaagccatgaaagccgggggtgcctgaagtccgtgaccgcgagggtcggcctagggtaaaaccggtgattggggctaagtcgtaacaaggtagccgtaccggaagg

SEQ ID NO: 31 - DNA, 1535 bp, Prevotella rara
ttttacagtggagagtttgatcctggctcaggatgaacgctagctacaggcttaacacatgcaagtcgcggggcagcatgaaggatgcttgcattctttgatggcgaccggcgcacgggtgagtaacgcgtatccaacctgcctgttaccacggcacagcccgtcgaaaggcggattaatgccgtatgtggtcttgaaagggcatctgatcatgactaaaggttcagcggtaacggatggggatgcgtccgattagctagacggcggggtaacggcccaccgtggcgacgatcggtaggggttctgagaggaaggtcccccacactggaactgagacacggtccagactcctacgggaggcagcagtgaggaatattggtcaatgggcgtaagcctgaaccagccaagtagcgtgagggaagactgccctatgggttgtaaacctcttttgtgcggggataaagtgagggacgtgtcccttattgcaggtaccgcacgaataaggaccggctaattccgtgccagcagccgcggtaatacggaaggtccgggcgttatccggatttattgggtttaaagggagcgcaggccgtcctttaagcgtgctgtgaaatgccgcggctcaaccgtggcactgcagcgcgaactggaggacttgagtacgcacgaggtaggcggaattcgtggtgtagcggtgaaatgcttagatatcacgaagaactccgattgcgaaggcagcttaccggagcgcaactgacgctgaggctcgaaagcgcgggtatcgaacaggattagataccctggtagtccgcgcggtaaacgatggatgcccgccgttgggatattgatttcagcggccaagcgaaagcgttaagcatcccacctggggagtacgccggcaacggtgaaactcaaaggaattgacgggggcccgcacaagcggaggaacatgtggtttaattcgatgatacgcgaggaaccttacccgggcttgaattgcaggagaacgatccagagatggtgaggcccttcggggctcctgtgaaggtgctgcatggttgtcgtcagctcgtgccgtgaggtgtcggctcaagtgccataacgagcgcaacccctgtccatagttgccatcaggtttgctgggcactctgtggagactgccgccgtaaggtgtgaggaaggtggggatgacgtcaaatcagcacggcccttacgtccggggctacacacgtgttacaatggggcatacagcgagttggatgtgcgcaagtacgtccggatcaataaagtgcctctcagttcggactggggtctgcaacccgaccccacgaagctggattcgctagtaatcgcgcatcagccatggcgcggtgaatacgttcccgggccttgtacacaccgcccgtcaagccatgaaagccgggggcgcctgaagtccgtgaccgcgagggtcggcctagggtgaaaccggtgattggggctaagtcgtaacaaggtagccgtaccggaaggtgcggctggaacacctcctttct

SEQ ID NO: 32 - DNA, 1438 bp, Prevotella rodentium
tgatggcgaccggcgcacgggtgagtaacgcgtatccaacctgccctttactatgggacagcccgtcgaaaggcggattaataccgtatgttgtcatgttgatgcatattttcatgaccaaaggcttcggccggtaaaggatggggatgcgtctgattagcttgccggcggggtaacggcccaccggggcgacgatcagtaggggttctgagaggaaggtcccccacattggaactgagacacggtccaaactcctacgggaggcagcagtgaggaatattggtcaatgggcgcgagcctgaaccagccaagtagcgtgcaggacgacggccctatgggttgtaaactgcttttatacggggataaagtatgccacgtgtggtttattgcaggtaccgtatgaataaggaccggctaattccgtgccagcagccgcggtaatacggaaggtccgggcgttatccggatttattgggtttaaagggagcgtaggccgggttttaagcgtgccgtgaaatgtcggggctcaaccttgacactgcggcgcgaactggagtccttgagtgcgcggaacgtatgcggaattcgtggtgtagcggtgaaatgcttagatatcacgaagaaccccgattgcgaaggcagcatacggcagcgctactgacgctgaagctcgaaggcgcgggtatcgaacaggattagataccctggtagtccgcgcggtaaacgatggatgcccgctgttggcgatatattgtcagcggccaagcgaaagcgttaagcatcccacctggggagtacgccggcaacggtgaaactcaaaggaattgacgggggcccgcacaagcggaggaacatgtggtttaattcgatgatacgcgaggaaccttacccgggcttgaactgccggcgaacgatccagagatggtgaggcccttcggggcgccggcggaggtgctgcatggttgtcgtcagctcgtgccgtgaggtgtcggcttaagtgccataacgagcgcaacccctgttctcagttgccatcgggtaatgccgggcactctgtgaagactgcctccgtaaggagtgaggagggtggggatgacgtcaaatcagcacggcccttacgtccggggctacacacgtgttacaatgggtggtacagacggtcggcgtccggcaacgtacgtccaatccgtaaagccgccctcagttcggactggggtctgcaacccgaccccacgaagctggattcgctagtaatcgcgcatcagccatggcgcggtgaatacgttcccgggccttgtacacaccgcccgtcaagccatgaaagccgggggcgcctgaagtccgtgaccgcgagggtcggcctagggtgaaaccggtgattggggctaagtcgtaacaaggtagccgtaccggaaggtgcggctggaacacctccttt

SEQ ID NO: 33 - DNA, 1531 bp, Prevotella muris
acaatgtagagtttgatcctggctcaggatgaacgctggctacaggcttaacacatgcaagtcgaggggcagcatgacatgttttcggacgtgtcgatggcgaccggcgcacgggtgagtaacgcgtatccgacctgccccgtaccagggcacagcccgtcgaaagacggattaatgccctatgttctccggaagatccatgttttccggagcaaaggttattccggtacgggatggggatgcgtccgattagcttgctggcggggtaacggcccaccagggcaccgatcggtaggggttctgagaggaaggtcccccacactggaactgagacacggtccagactcctacgggaggcagcagtgaggaatattggtcaatggggggaaccctgaaccagccaagtagcgtgcaggatgacggccctatgggttgtaaactgcttttgtgcgtggataaagtaggccacttgtggccttttgcaggtaccgcacgaataaggaccggctaattccgtgccagcagccgcggtaatacggaaggtccgggcgttatccggatttattgggtttaaagggagcgtaggccgcctgtcaagcgtgctgtgaaacgccgtggctcaaccacggtcctgcagcgcgaactggcgggcttgagtgtgcggaaggcacgcggaattcgtggtgtagcggtgaaatgcttagatatcacgaagaactccgattgcgaaggcagcgtgccgcagcattactgacgctgatgctcgaaagcgcgggtatcgaacaggattagataccctggtagtccgcgcggtaaacgatggatgcccgctgtcggcgatatacagtcggcggccaagcgaaagcgttaagcatcccacctggggagtacgccggcaacggtgaaactcaaaggaattgacgggggcccgcacaagcggaggaacatgtggtttaattcgatgatacgcgaggaaccttacccgggcttgaattgcagatgaatgattcagagatgatgaagtccttcgggacatctgtgaaggtgctgcatggttgtcgtcagctcgtgccgtgaggtgtcggcttaagtgccataacgagcgcaaccccttccctcagttgccatcgggtcatgccgggcactctgtgggtactgcctccgcaaggagcgaggaaggcggggatgacgtcaaatcagcacggcccttacgtccggggctacacacgtgttacaatggggcatacagcgagcaggtgccgtgcaaacggtgtcgaatcttgaaagtgcccctcagttcggactggggtctgcaacccgaccccacgaagctggattcgctagtaatcgcgcatcagccatggcgcggtgaatacgttcccgggccttgtacacaccgcccgtcaagccatgaaagccgggggcgcctgaagtccgtgaccgtgagggtcggcctagggtgaaaccggtgattggggctaagtcgtaacaaggtagccgtaccggaaggtgcggctggaacacctccttt

SEQ ID NO: 34 - protein, 5 aa, Artificial Sequence
  Synthesized oligonucleotide
GGGGS

SEQ ID NO: 35 - DNA, 24 bp, Artificial Sequence
  Synthesized oligonucleotide
gtcgtggagtctactggtgtcttc

SEQ ID NO: 36 - DNA, 24 bp, Artificial Sequence
  Synthesized oligonucleotide
gtcatatttctcgtggttcacacc

SEQ ID NO: 37 - DNA, 20 bp, Artificial Sequence
  Synthesized oligonucleotide
tgtgaccctcaatgccagag

SEQ ID NO: 38 - DNA, 19 bp, Artificial Sequence
  Synthesized oligonucleotide
agcactggggcatcaacac

SEQ ID NO: 39 - DNA, 20 bp, Artificial Sequence
  Synthesized oligonucleotide
agrgtttgatymtggctcag

SEQ ID NO: 40 - DNA, 22 bp, Artificial Sequence
  Synthesized oligonucleotide
tacggytaccttgttacgactt

SEQ ID NO: 41 - DNA, 90 bp, Artificial Sequence
  Synthesized oligonucleotide
  misc_feature (30)..(37): n is a, c, g, or t
aatgatacggcgaccaccgagatctacacnnnnnnnnacactctttccctacacgacgctcttccgatctagrgtttgatymtggctcag

SEQ ID NO: 42 - DNA, 85 bp, Artificial Sequence
  Synthesized oligonucleotide
  misc_feature (25)..(32): n is a, c, g, or t
caagcagaagacggcatacgagatnnnnnnnngtgactggagttcagacgtgtgctcttccgatcttgctgcctcccgtaggagt

SEQ ID NO: 43 - DNA, 20 bp, Artificial Sequence
  Synthesized oligonucleotide
cgtaggagtttggaccgtgt

SEQ ID NO: 44 - DNA, 20 bp, Artificial Sequence
  Synthesized oligonucleotide
gcatgggagcgacaaataaa

SEQ ID NO: 45 - DNA, 21 bp, Artificial Sequence
  Synthesized oligonucleotide
aagagtgattggcgtccgtac

SEQ ID NO: 46 - DNA, 21 bp, Artificial Sequence
  Synthesized oligonucleotide
atggacacgtcactggcagag

SEQ ID NO: 47 - DNA, 38 bp, Artificial Sequence
  Synthesized oligonucleotide
gtggatcccccgggctgcagcatccctcctccatctgt

SEQ ID NO: 48 - DNA, 39 bp, Artificial Sequence
  Synthesized oligonucleotide
ctggaagataggcaattagtttgggacgtaggggcaatc

SEQ ID NO: 49 - DNA, 27 bp, Artificial Sequence
  Synthesized oligonucleotide
tcccgaccgactgatcctttttaaccc

SEQ ID NO: 50 - DNA, 20 bp, Artificial Sequence
  Synthesized oligonucleotide
ctgtgcccagtaattttgtg

SEQ ID NO: 51 - DNA, 39 bp, Artificial Sequence
  Synthesized oligonucleotide
gtggatcccccgggctgcaccccttgtccatgttagacg

SEQ ID NO: 52 - DNA, 39 bp, Artificial Sequence
  Synthesized oligonucleotide
ctggaagataggcaattagtgaagtgacaggggatgcta

SEQ ID NO: 53 - DNA, 33 bp, Artificial Sequence
  Synthesized oligonucleotide
aaacaaataaatgaagaaaattttatctttgct

SEQ ID NO: 54 - DNA, 39 bp, Artificial Sequence; identical to SEQ ID NO: 52
  Synthesized oligonucleotide

SEQ ID NO: 55 - DNA, 39 bp, Artificial Sequence
  Synthesized oligonucleotide
gtggatcccccgggctgcaacactgatgtcgttgccttt

SEQ ID NO: 56 - DNA, 39 bp, Artificial Sequence
  Synthesized oligonucleotide
ctggaagataggcaattaggcaaccttaccacagggaaa

SEQ ID NO: 57 - DNA, 33 bp, Artificial Sequence; identical to SEQ ID NO: 53
  Synthesized oligonucleotide

SEQ ID NO: 58 - DNA, 39 bp, Artificial Sequence; identical to SEQ ID NO: 56
  Synthesized oligonucleotide

SEQ ID NO: 59 - DNA, 39 bp, Artificial Sequence
  Synthesized oligonucleotide
gtggatcccccgggctgcacaagtagagttccggttcgg

SEQ ID NO: 60 - DNA, 39 bp, Artificial Sequence
  Synthesized oligonucleotide
ctggaagataggcaattagaaatcacgaccctcgatgtg

SEQ ID NO: 61 - DNA, 33 bp, Artificial Sequence; identical to SEQ ID NO: 53
  Synthesized oligonucleotide

SEQ ID NO: 62 - DNA, 39 bp, Artificial Sequence; identical to SEQ ID NO: 60
  Synthesized oligonucleotide

SEQ ID NO: 63 - DNA, 39 bp, Artificial Sequence
  Synthesized oligonucleotide
gtggatcccccgggctgcaagttcgttcttctcgatggc

SEQ ID NO: 64 - DNA, 39 bp, Artificial Sequence
  Synthesized oligonucleotide
ctggaagataggcaattagcaaccgcgggtataacaaga

SEQ ID NO: 65 - DNA, 33 bp, Artificial Sequence; identical to SEQ ID NO: 53
  Synthesized oligonucleotide

SEQ ID NO: 66 - DNA, 39 bp, Artificial Sequence; identical to SEQ ID NO: 64
  Synthesized oligonucleotide

SEQ ID NO: 67 - DNA, 39 bp, Artificial Sequence
  Synthesized oligonucleotide
gtggatcccccgggctgcatggggcgtttgtatttgtca

SEQ ID NO: 68 - DNA, 39 bp, Artificial Sequence
  Synthesized oligonucleotide
ctggaagataggcaattagaaaccgctgacggtctattc

SEQ ID NO: 69 - DNA, 33 bp, Artificial Sequence; identical to SEQ ID NO: 53
  Synthesized oligonucleotide

SEQ ID NO: 70 - DNA, 39 bp, Artificial Sequence; identical to SEQ ID NO: 68
  Synthesized oligonucleotide

SEQ ID NO: 71 - DNA, 39 bp, Artificial Sequence
  Synthesized oligonucleotide
gtggatcccccgggctgcatccagtcgtcagactttcct

SEQ ID NO: 72 - DNA, 39 bp, Artificial Sequence
  Synthesized oligonucleotide
ctggaagataggcaattaggaagggactaaaatcgccgt

SEQ ID NO: 73 - DNA, 33 bp, Artificial Sequence; identical to SEQ ID NO: 53
  Synthesized oligonucleotide

SEQ ID NO: 74 - DNA, 39 bp, Artificial Sequence; identical to SEQ ID NO: 72
  Synthesized oligonucleotide

SEQ ID NO: 75 - DNA, 39 bp, Artificial Sequence
  Synthesized oligonucleotide
gtggatcccccgggctgcagggtcgcttacattttgcac

SEQ ID NO: 76 - DNA, 39 bp, Artificial Sequence
  Synthesized oligonucleotide
ctggaagataggcaattagtcggtgattatgctttcgca

SEQ ID NO: 77 - DNA, 33 bp, Artificial Sequence; identical to SEQ ID NO: 53
  Synthesized oligonucleotide

SEQ ID NO: 78 - DNA, 39 bp, Artificial Sequence; identical to SEQ ID NO: 76
  Synthesized oligonucleotide

SEQ ID NO: 79 - DNA, 39 bp, Artificial Sequence
  Synthesized oligonucleotide
gtggatcccccgggctgcacttgcttcaaatcacgctgg

SEQ ID NO: 80 - DNA, 39 bp, Artificial Sequence
  Synthesized oligonucleotide
ctggaagataggcaattaggttgcgtaatgtgaacggtg

SEQ ID NO: 81 - DNA, 33 bp, Artificial Sequence; identical to SEQ ID NO: 53
  Synthesized oligonucleotide

SEQ ID NO: 82 - DNA, 39 bp, Artificial Sequence; identical to SEQ ID NO: 80
  Synthesized oligonucleotide

SEQ ID NO: 83 - DNA, 39 bp, Artificial Sequence
  Synthesized oligonucleotide
gtggatcccccgggctgcatgtcgaaaggcatcatctgg

SEQ ID NO: 84 - DNA, 39 bp, Artificial Sequence
  Synthesized oligonucleotide
ctggaagataggcaattagaccattacggccattaccac

SEQ ID NO: 85 - DNA, 33 bp, Artificial Sequence; identical to SEQ ID NO: 53
  Synthesized oligonucleotide

SEQ ID NO: 86 - DNA, 39 bp, Artificial Sequence; identical to SEQ ID NO: 84
  Synthesized oligonucleotide

SEQ ID NO: 87 - DNA, 39 bp, Artificial Sequence
  Synthesized oligonucleotide
gtggatcccccgggctgcagtgccagtttcaaccaatcg

SEQ ID NO: 88 - DNA, 39 bp, Artificial Sequence
  Synthesized oligonucleotide
ctggaagataggcaattagcttgtaccccagcagatgtc

SEQ ID NO: 89 - DNA, 33 bp, Artificial Sequence; identical to SEQ ID NO: 53
  Synthesized oligonucleotide

SEQ ID NO: 90 - DNA, 39 bp, Artificial Sequence
  Synthesized oligonucleotide
ctggaagataggcaattaggtaagctggcgcttgaaatc

SEQ ID NO: 91 - DNA, 39 bp, Artificial Sequence
  Synthesized oligonucleotide
gtggatcccccgggctgcattgttttggttgtaactgcc

SEQ ID NO: 92 - DNA, 39 bp, Artificial Sequence
  Synthesized oligonucleotide
ctggaagataggcaattaggtcaatacgaactgcaactg

SEQ ID NO: 93 - DNA, 33 bp, Artificial Sequence; identical to SEQ ID NO: 53
  Synthesized oligonucleotide

SEQ ID NO: 94 - DNA, 39 bp, Artificial Sequence; identical to SEQ ID NO: 92
  Synthesized oligonucleotide

SEQ ID NO: 95 - DNA, 39 bp, Artificial Sequence
  Synthesized oligonucleotide
gtggatcccccgggctgcagaccaattaagcacgtcaag

SEQ ID NO: 96 - DNA, 39 bp, Artificial Sequence
  Synthesized oligonucleotide
ctggaagataggcaattagtggtacaattcgctcaaaga

SEQ ID NO: 97 - DNA, 33 bp, Artificial Sequence; identical to SEQ ID NO: 53
  Synthesized oligonucleotide

SEQ ID NO: 98 - DNA, 39 bp, Artificial Sequence; identical to SEQ ID NO: 96
  Synthesized oligonucleotide

SEQ ID NO: 99 - DNA, 39 bp, Artificial Sequence
  Synthesized oligonucleotide
gtggatcccccgggctgcatactcccgtgtttttagtgg

SEQ ID NO: 100 - DNA, 39 bp, Artificial Sequence
  Synthesized oligonucleotide
ctggaagataggcaattagggatgccagttacctgatag

SEQ ID NO: 101 - DNA, 33 bp, Artificial Sequence; identical to SEQ ID NO: 53
  Synthesized oligonucleotide

SEQ ID NO: 102 - DNA, 39 bp, Artificial Sequence; identical to SEQ ID NO: 100
  Synthesized oligonucleotide

SEQ ID NO: 103 - DNA, 39 bp, Artificial Sequence
  Synthesized oligonucleotide
gtggatcccccgggctgcatcaaaccacacacagagaaa

SEQ ID NO: 104 - DNA, 39 bp, Artificial Sequence
  Synthesized oligonucleotide
ctggaagataggcaattaggaattcggccaaaccttatg

SEQ ID NO: 105 - DNA, 33 bp, Artificial Sequence; identical to SEQ ID NO: 53
  Synthesized oligonucleotide

SEQ ID NO: 106 - DNA, 39 bp, Artificial Sequence; identical to SEQ ID NO: 104
  Synthesized oligonucleotide

SEQ ID NO: 107 - DNA, 39 bp, Artificial Sequence
  Synthesized oligonucleotide
gtggatcccccgggctgcaagacaatcgaggcatcatac

SEQ ID NO: 108 - DNA, 39 bp, Artificial Sequence
  Synthesized oligonucleotide
ctggaagataggcaattagatagcgtgaatggaaaacct

SEQ ID NO: 109 - DNA, 33 bp, Artificial Sequence; identical to SEQ ID NO: 53
  Synthesized oligonucleotide

SEQ ID NO: 110 - DNA, 39 bp, Artificial Sequence; identical to SEQ ID NO: 108
  Synthesized oligonucleotide

SEQ ID NO: 111 - DNA, 39 bp, Artificial Sequence
  Synthesized oligonucleotide
gtggatcccccgggctgcaatctatctcaacctcctgct

SEQ ID NO: 112 - DNA, 39 bp, Artificial Sequence
  Synthesized oligonucleotide
ctggaagataggcaattaggaaggaatcagcgtagatgt

SEQ ID NO: 113 - DNA, 33 bp, Artificial Sequence; identical to SEQ ID NO: 53
  Synthesized oligonucleotide

SEQ ID NO: 114 - DNA, 39 bp, Artificial Sequence; identical to SEQ ID NO: 112
  Synthesized oligonucleotide

SEQ ID NO: 115 - DNA, 39 bp, Artificial Sequence
  Synthesized oligonucleotide
gtggatcccccgggctgcatgtgccgataacctgaatgg

SEQ ID NO: 116 - DNA, 39 bp, Artificial Sequence
  Synthesized oligonucleotide
ctggaagataggcaattagcagagaaaagggctggtgtt

SEQ ID NO: 117 - DNA, 33 bp, Artificial Sequence; identical to SEQ ID NO: 53
  Synthesized oligonucleotide

SEQ ID NO: 118 - DNA, 39 bp, Artificial Sequence; identical to SEQ ID NO: 116
  Synthesized oligonucleotide

SEQ ID NO: 119 - DNA, 30 bp, Artificial Sequence
  Synthesized oligonucleotide
tcccgaccgaggtctttgtccccttctccg

SEQ ID NO: 120 - DNA, 30 bp, Artificial Sequence
  Synthesized oligonucleotide
tcttacaccggcgggttgctttttatgcct

SEQ ID NO: 121 - DNA, 20 bp, Artificial Sequence
  Synthesized oligonucleotide
gcctgatgcatggaaaaacc

SEQ ID NO: 122 - DNA, 19 bp, Artificial Sequence
  Synthesized oligonucleotide
ctggaagataggcaattag

SEQ ID NO: 123 - DNA, 39 bp, Artificial Sequence
  Synthesized oligonucleotide
gtggatcccccgggctgcacggataacggaattacccat

SEQ ID NO: 124 - DNA, 39 bp, Artificial Sequence
  Synthesized oligonucleotide
ctggaagataggcaattagtctgacaaaggttggttgaa

SEQ ID NO: 125 - DNA, 33 bp, Artificial Sequence; identical to SEQ ID NO: 53
  Synthesized oligonucleotide

SEQ ID NO: 126 - DNA, 39 bp, Artificial Sequence; identical to SEQ ID NO: 124
  Synthesized oligonucleotide

SEQ ID NO: 127 - DNA, 39 bp, Artificial Sequence
  Synthesized oligonucleotide
gtggatcccccgggctgcatgtataacccccagaaggaa

SEQ ID NO: 128 - DNA, 39 bp, Artificial Sequence
  Synthesized oligonucleotide
ctggaagataggcaattagaacaataccgtcaacctctc

SEQ ID NO: 129 - DNA, 33 bp, Artificial Sequence; identical to SEQ ID NO: 53
  Synthesized oligonucleotide

SEQ ID NO: 130 - DNA, 39 bp, Artificial Sequence; identical to SEQ ID NO: 128
  Synthesized oligonucleotide

SEQ ID NO: 131 - DNA, 39 bp, Artificial Sequence
  Synthesized oligonucleotide
gtggatcccccgggctgcatttattagccgtggtatcgg

SEQ ID NO: 132 - DNA, 39 bp, Artificial Sequence
  Synthesized oligonucleotide
ctggaagataggcaattagactccaacagcatcttcaat

SEQ ID NO: 133 - DNA, 33 bp, Artificial Sequence; identical to SEQ ID NO: 53
  Synthesized oligonucleotide

SEQ ID NO: 134 - DNA, 39 bp, Artificial Sequence; identical to SEQ ID NO: 132
  Synthesized oligonucleotide

SEQ ID NO: 135 - DNA, 39 bp, Artificial Sequence
  Synthesized oligonucleotide
gtggatcccccgggctgcagtagtgtatcgctttgtcct

SEQ ID NO: 136 - DNA, 39 bp, Artificial Sequence
  Synthesized oligonucleotide
ctggaagataggcaattagattcattactggtcggaacc

SEQ ID NO: 137 - DNA, 33 bp, Artificial Sequence; identical to SEQ ID NO: 53
  Synthesized oligonucleotide

SEQ ID NO: 138 - DNA, 39 bp, Artificial Sequence; identical to SEQ ID NO: 136
  Synthesized oligonucleotide

SEQ ID NO: 139 - DNA, 39 bp, Artificial Sequence
  Synthesized oligonucleotide
gtggatcccccgggctgcagggatactgaatgtctgtcc

SEQ ID NO: 140 - DNA, 39 bp, Artificial Sequence
  Synthesized oligonucleotide
ctggaagataggcaattagacagtgtaatcatcaacgct

SEQ ID NO: 141 - DNA, 33 bp, Artificial Sequence; identical to SEQ ID NO: 53
  Synthesized oligonucleotide

SEQ ID NO: 142 - DNA, 39 bp, Artificial Sequence; identical to SEQ ID NO: 140
  Synthesized oligonucleotide

SEQ ID NO: 143 - DNA, 39 bp, Artificial Sequence
  Synthesized oligonucleotide
gtggatcccccgggctgcaattttcaatccagtccctcc

SEQ ID NO: 144 - DNA, 39 bp, Artificial Sequence
  Synthesized oligonucleotide
ctggaagataggcaattagtacagtttgccgataccaaa

SEQ ID NO: 145 - DNA, 33 bp, Artificial Sequence; identical to SEQ ID NO: 53
  Synthesized oligonucleotide

SEQ ID NO: 146 - DNA, 39 bp, Artificial Sequence; identical to SEQ ID NO: 144
  Synthesized oligonucleotide

SEQ ID NO: 147 - DNA, 39 bp, Artificial Sequence
  Synthesized oligonucleotide
gtggatcccccgggctgcatatgaactacaaagtcatcg

SEQ ID NO: 148 - DNA, 27 bp, Artificial Sequence
  Synthesized oligonucleotide
ttcaagaagcaccaccgttatgatata

SEQ ID NO: 149 - DNA, 27 bp, Artificial Sequence
  Synthesized oligonucleotide
taacggtggtgcttcttgaaaattaag

SEQ ID NO: 150 - DNA, 35 bp, Artificial Sequence
  Synthesized oligonucleotide
ctggaagataggcaattaggacgatttcgtggaca

SEQ ID NO: 151 - DNA, 39 bp, Artificial Sequence; identical to SEQ ID NO: 147
  Synthesized oligonucleotide

SEQ ID NO: 152 - DNA, 35 bp, Artificial Sequence; identical to SEQ ID NO: 150
  Synthesized oligonucleotide

SEQ ID NO: 153 - DNA, 19 bp, Artificial Sequence
  Synthesized oligonucleotide
tcaacgcaccattactttc

SEQ ID NO: 154 - DNA, 20 bp, Artificial Sequence
  Synthesized oligonucleotide
atgaaaaacagtttacttgc

SEQ ID NO: 155 - DNA, 39 bp, Artificial Sequence
  Synthesized oligonucleotide
gtggatcccccgggctgcatacaatccgttggaactgtc

SEQ ID NO: 156 - DNA, 30 bp, Artificial Sequence
  Synthesized oligonucleotide
attagtatttcagcattcatttgctggtga

SEQ ID NO: 157 - DNA, 40 bp, Artificial Sequence
  Synthesized oligonucleotide
atgaatgctgaaatactaattttagatagactataatttg

SEQ ID NO: 158 - DNA, 39 bp, Artificial Sequence
  Synthesized oligonucleotide
ctggaagataggcaattaggaactggtcgtaaaaatcac

SEQ ID NO: 159 - DNA, 39 bp, Artificial Sequence; identical to SEQ ID NO: 155
  Synthesized oligonucleotide

SEQ ID NO: 160 - DNA, 39 bp, Artificial Sequence; identical to SEQ ID NO: 158
  Synthesized oligonucleotide

SEQ ID NO: 161 - DNA, 39 bp, Artificial Sequence; identical to SEQ ID NO: 71
  Synthesized oligonucleotide

SEQ ID NO: 162 - DNA, 39 bp, Artificial Sequence; identical to SEQ ID NO: 72
  Synthesized oligonucleotide

SEQ ID NO: 163 - DNA, 39 bp, Artificial Sequence
  Synthesized oligonucleotide
gtggatcccccgggctgcaatccttccacttttcctctc

SEQ ID NO: 164 - DNA, 30 bp, Artificial Sequence
  Synthesized oligonucleotide
aattgatcgttctaaagccgacgatttaag

SEQ ID NO: 165 - DNA, 35 bp, Artificial Sequence
  Synthesized oligonucleotide
cggctttagaacgatcaattttaaaatgaatatat

SEQ ID NO: 166 - DNA, 39 bp, Artificial Sequence
  Synthesized oligonucleotide
ctggaagataggcaattagttcaacgaaaacagaacatc

SEQ ID NO: 167 - DNA, 39 bp, Artificial Sequence; identical to SEQ ID NO: 163
  Synthesized oligonucleotide

SEQ ID NO: 168 - DNA, 39 bp, Artificial Sequence; identical to SEQ ID NO: 166
  Synthesized oligonucleotide

SEQ ID NO: 169 - DNA, 39 bp, Artificial Sequence; identical to SEQ ID NO: 107
  Synthesized oligonucleotide

SEQ ID NO: 170 - DNA, 39 bp, Artificial Sequence; identical to SEQ ID NO: 108
  Synthesized oligonucleotide

SEQ ID NO: 171 - DNA, 30 bp, Artificial Sequence
  Synthesized oligonucleotide
attcgtaaaacaccaccaccaccaccactg

SEQ ID NO: 172 - DNA, 30 bp, Artificial Sequence
  Synthesized oligonucleotide
tcacgccgtccatggtatatctccttctta

SEQ ID NO: 173 - DNA, 30 bp, Artificial Sequence
  Synthesized oligonucleotide
atataccatggacggcgtgagccaacctac

SEQ ID NO: 174 - DNA, 30 bp, Artificial Sequence
  Synthesized oligonucleotide
ggtggtggtgttttacgaatactttcttca

SEQ ID NO: 175 - DNA, 30 bp, Artificial Sequence
  Synthesized oligonucleotide
gatggtaaaacaccaccaccaccaccactg

SEQ ID NO: 176 - DNA, 30 bp, Artificial Sequence
  Synthesized oligonucleotide
cttcaccaaccatggtatatctccttctta

SEQ ID NO: 177 - DNA, 30 bp, Artificial Sequence
  Synthesized oligonucleotide
atataccatggttggtgaagatttacattt

SEQ ID NO: 178 - DNA, 30 bp, Artificial Sequence
  Synthesized oligonucleotide
ggtggtggtgttttaccatcatcttcttac